European Patent Application EP 4 527 931 A1, published March 26, 2025. Title: Methods and Compositions for Editing RNAs. Applicant: Peking University. The sequence listing filed with the application follows.

SEQUENCE LISTING (400 sequences)

SEQ ID NO: 1 - DNA, 708 bp, synthetic construct
  source 1..708: mol_type = other DNA
atggtgagcaagggcgaggaggataacatggccatcatcaaggagttcatgcgcttcaaggtgcacatggagggctccgtgaacggccacgagttcgagatcgagggcgagggcgagggccgcccctacgagggcacccagaccgccaagctgaaggtgaccaagggtggccccctgcccttcgcctgggacatcctgtcccctcagttcatgtacggctccaaggcctacgtgaagcaccccgccgacatccccgactacttgaagctgtccttccccgagggcttcaagtgggagcgcgtgatgaacttcgaggacggcggcgtggtgaccgtgacccaggactcctccctgcaggacggcgagttcatctacaaggtgaagctgcgcggcaccaacttcccctccgacggccccgtaatgcagaagaagaccatgggctgggaggcctcctccgagcggatgtaccccgaggacggcgccctgaagggcgagatcaagcagaggctgaagctgaaggacggcggccactacgacgctgaggtcaagaccacctacaaggccaagaagcccgtgcagctgcccggcgcctacaacgtcaacatcaagttggacatcacctcccacaacgaggactacaccatcgtggaacagtacgaacgcgccgagggccgccactccaccggcggcatggacgagctgtacaag

SEQ ID NO: 2 - DNA, 99 bp, synthetic construct
  source 1..99: mol_type = other DNA
ctgcagggcggaggaggcagcggcggaggaggcagcggcggaggaggcagcagaaggtatacacgccggaagaatctgtagagatccccggtcgccacc

SEQ ID NO: 3 - DNA, 717 bp, synthetic construct
  source 1..717: mol_type = other DNA
gtgagcaagggcgaggagctgttcaccggggtggtgcccatcctggtcgagctggacggcgacgtaaacggccacaagttcagcgtgtccggcgagggcgagggcgatgccacctacggcaagctgaccctgaagttcatctgcaccaccggcaagctgcccgtgccctggcccaccctcgtgaccaccctgacctacggcgtgcagtgcttcagccgctaccccgaccacatgaagcagcacgacttcttcaagtccgccatgcccgaaggctacgtccaggagcgcaccatcttcttcaaggacgacggcaactacaagacccgcgccgaggtgaagttcgagggcgacaccctggtgaaccgcatcgagctgaagggcatcgacttcaaggaggacggcaacatcctggggcacaagctggagtacaactacaacagccacaacgtctatatcatggccgacaagcagaagaacggcatcaaggtgaacttcaagatccgccacaacatcgaggacggcagcgtgcagctcgccgaccactaccagcagaacacccccatcggcgacggccccgtgctgctgcccgacaaccactacctgagcacccagtccgccctgagcaaagaccccaacgagaagcgcgatcacatggtcctgctggagttcgtgaccgccgccgggatcactctcggcatggacgagctgtacaagtaa

SEQ ID NO: 4 - DNA, 81 bp, synthetic construct
  source 1..81: mol_type = other DNA
ctgcagggcggaggaggcagcggcggaggaggcagcggcggaggaggcagcgcctgctcgcgatgctagagggctctgcca

SEQ ID NO: 5 - DNA, 51 bp, synthetic construct
  source 1..51: mol_type = other DNA
ctgcagggcggaggaggcagcgcctgctcgcgatgctagagggctctgcca

SEQ ID NO: 6 - RNA, 101 nt, synthetic construct
  misc_feature 1..101: note = synthesized sequence
  source 1..101: mol_type = other RNA
ggaccaccccaaaaatgaatataaccaaaactgaacagctcctcgcccttgctcactggcagagccctccagcatcgcgagcaggcgctgcctcctccgcc

SEQ ID NO: 7 - RNA, 70 nt, synthetic construct
  misc_feature 1..70: note = synthesized sequence
  source 1..70: mol_type = other RNA
aaaccgagggatcataggggactgaatccaccattcttctcccaatccctgcaactccttcttcccctgc

SEQ ID NO: 8 - RNA, 70 nt, synthetic construct
  misc_feature 1..70: note = synthesized sequence
  source 1..70: mol_type = other RNA
tgaacagctcctcgcccttgctcactggcagagccctccagcatcgcgagcaggcgctgcctcctccgcc

SEQ ID NO: 9 - DNA, 111 bp, synthetic construct
  misc_feature 1..111: note = synthesized sequence
  source 1..111: mol_type = other DNA
atggacgagctgtacaagctgcagggcggaggaggcagcgcctgctcgcgatgctatagggctctgccagtgagcaagggcgaggagctgttcaccggggtggtgcccatc

SEQ ID NO: 10 - DNA, 111 bp, synthetic construct
  misc_feature 1..111: note = synthesized sequence
  source 1..111: mol_type = other DNA
atggacgagctgtacaagctgcagggcggaggaggcagcgcctgctcgcgatgctaaagggctctgccagtgagcaagggcgaggagctgttcaccggggtggtgcccatc

SEQ ID NO: 11 - DNA, 111 bp, synthetic construct
  misc_feature 1..111: note = synthesized sequence
  source 1..111: mol_type = other DNA
atggacgagctgtacaagctgcagggcggaggaggcagcgcctgctcgcgatgctacagggctctgccagtgagcaagggcgaggagctgttcaccggggtggtgcccatc

SEQ ID NO: 12 - DNA, 111 bp, synthetic construct
  misc_feature 1..111: note = synthesized sequence
  source 1..111: mol_type = other DNA
atggacgagctgtacaagctgcagggcggaggaggcagcgcctgctcgcgatgctagagggctctgccagtgagcaagggcgaggagctgttcaccggggtggtgcccatc

SEQ ID NO: 13 - DNA, 111 bp, synthetic construct
  misc_feature 1..111: note = synthesized sequence
  source 1..111: mol_type = other DNA
atggacgagctgtacaagctgcagggcggaggaggcagcgcctgctcgcgatgcaatagggctctgccagtgagcaagggcgaggagctgttcaccggggtggtgcccatc

SEQ ID NO: 14 - DNA, 111 bp, synthetic construct
  misc_feature 1..111: note = synthesized sequence
  source 1..111: mol_type = other DNA
atggacgagctgtacaagctgcagggcggaggaggcagcgcctgctcgcgatgcaaaagggctctgccagtgagcaagggcgaggagctgttcaccggggtggtgcccatc

SEQ ID NO: 15 - DNA, 111 bp, synthetic construct
  misc_feature 1..111: note = synthesized sequence
  source 1..111: mol_type = other DNA
atggacgagctgtacaagctgcagggcggaggaggcagcgcctgctcgcgatgcaacagggctctgccagtgagcaagggcgaggagctgttcaccggggtggtgcccatc

SEQ ID NO: 16 - DNA, 111 bp, synthetic construct
  misc_feature 1..111: note = synthesized sequence
  source 1..111: mol_type = other DNA
atggacgagctgtacaagctgcagggcggaggaggcagcgcctgctcgcgatgcaagagggctctgccagtgagcaagggcgaggagctgttcaccggggtggtgcccatc

SEQ ID NO: 17 - DNA, 111 bp, synthetic construct
  misc_feature 1..111: note = synthesized sequence
  source 1..111: mol_type = other DNA
atggacgagctgtacaagctgcagggcggaggaggcagcgcctgctcgcgatgccatagggctctgccagtgagcaagggcgaggagctgttcaccggggtggtgcccatc

SEQ ID NO: 18 - DNA, 111 bp, synthetic construct
  misc_feature 1..111: note = synthesized sequence
  source 1..111: mol_type = other DNA
atggacgagctgtacaagctgcagggcggaggaggcagcgcctgctcgcgatgccaaagggctctgccagtgagcaagggcgaggagctgttcaccggggtggtgcccatc

SEQ ID NO: 19 - DNA, 111 bp, synthetic construct
  misc_feature 1..111: note = synthesized sequence
  source 1..111: mol_type = other DNA
atggacgagctgtacaagctgcagggcggaggaggcagcgcctgctcgcgatgccacagggctctgccagtgagcaagggcgaggagctgttcaccggggtggtgcccatc

SEQ ID NO: 20 - DNA, 111 bp, synthetic construct
  misc_feature 1..111: note = synthesized sequence
  source 1..111: mol_type = other DNA
atggacgagctgtacaagctgcagggcggaggaggcagcgcctgctcgcgatgccagagggctctgccagtgagcaagggcgaggagctgttcaccggggtggtgcccatc

SEQ ID NO: 21 - DNA, 111 bp, synthetic construct
  misc_feature 1..111: note = synthesized sequence
  source 1..111: mol_type = other DNA
atggacgagctgtacaagctgcagggcggaggaggcagcgcctgctcgcgatgcgatagggctctgccagtgagcaagggcgaggagctgttcaccggggtggtgcccatc

SEQ ID NO: 22 - DNA, 111 bp, synthetic construct
  misc_feature 1..111: note = synthesized sequence
  source 1..111: mol_type = other DNA
atggacgagctgtacaagctgcagggcggaggaggcagcgcctgctcgcgatgcgaaagggctctgccagtgagcaagggcgaggagctgttcaccggggtggtgcccatc

SEQ ID NO: 23 - DNA, 111 bp, synthetic construct
  misc_feature 1..111: note = synthesized sequence
  source 1..111: mol_type = other DNA
atggacgagctgtacaagctgcagggcggaggaggcagcgcctgctcgcgatgcgacagggctctgccagtgagcaagggcgaggagctgttcaccggggtggtgcccatc

SEQ ID NO: 24 - DNA, 111 bp, synthetic construct
  misc_feature 1..111: note = synthesized sequence
  source 1..111: mol_type = other DNA
atggacgagctgtacaagctgcagggcggaggaggcagcgcctgctcgcgatgcgagagggctctgccagtgagcaagggcgaggagctgttcaccggggtggtgcccatc

SEQ ID NO: 25 - RNA, 91 nt, synthetic construct
  misc_feature 1..91: note = synthesized sequence
  source 1..91: mol_type = other RNA
tagctgtatcgtcaaggcactcttgcctacgccaccagctccaaccaccacaagtttatattcagtcattttcagcaggcctctctcccgc

SEQ ID NO: 26 - RNA, 111 nt, synthetic construct
  misc_feature 1..111: note = synthesized sequence
  source 1..111: mol_type = other RNA
gattctgaattagctgtatcgtcaaggcactcttgcctacgccaccagctccaactaccacaagtttatattcagtcattttcagcaggcctctctcccgcacctgggagc

SEQ ID NO: 27 - RNA, 131 nt, synthetic construct
  misc_feature 1..131: note = synthesized sequence
  source 1..131: mol_type = other RNA
tccacaaaatgattctgaattagctgtatcgtcaaggcactcttgcctacgccaccagctccaactaccacaagtttatattcagtcattttcagcaggcctctctcccgcacctgggagccgctgagcct

SEQ ID NO: 28 - RNA, 151 nt, synthetic construct
  misc_feature 1..151: note = synthesized sequence
  source 1..151: mol_type = other RNA
atcatattcgtccacaaaatgattctgaattagctgtatcgtcaaggcactcttgcctacgccaccagctccaaccaccacaagtttatattcagtcattttcagcaggcctctctcccgcacctgggagccgctgagcctctggccccgc

SEQ ID NO: 29 - RNA, 171 nt, synthetic construct
  misc_feature 1..171: note = synthesized sequence
  source 1..171: mol_type = other RNA
ctattgttggatcatattcgtccacaaaatgattctgaattagctgtatcgtcaaggcactcttgcctacgccaccagctccaaccaccacaagtttatattcagtcattttcagcaggcctctctcccgcacctgggagccgctgagcctctggccccgccgccgccttc

SEQ ID NO: 30 - RNA, 191 nt, synthetic construct
  misc_feature 1..191: note = synthesized sequence
  source 1..191: mol_type = other RNA
taggaatcctctattgttggatcatattcgtccacaaaatgattctgaattagctgtatcgtcaaggcactcttgcctacgccaccagctccaaccaccacaagtttatattcagtcattttcagcaggcctctctcccgcacctgggagccgctgagcctctggccccgccgccgccttcagtgcctgcg

SEQ ID NO: 31 - RNA, 151 nt, synthetic construct
  misc_feature 1..151: note = synthesized sequence
  source 1..151: mol_type = other RNA
gaggcgcagcatccacaggcggaggcgaaagcagcccggacagctgaggccggaagagggtggggccgcggtggccagggagccggcgccgccacgcgcgggtgggggggactggggttgctcgcgggctccgggcgggcggcgggcgccg

SEQ ID NO: 32 - RNA, 151 nt, synthetic construct
  misc_feature 1..151: note = synthesized sequence
  source 1..151: mol_type = other RNA
tcctgtagctaaggccacaaaattatccactgtttttggaacagtctttccgaagagaccaaagatcacccggcccacatcttcatctccaattcgtaggtcaaaatacaccttgacggtgactttgggccccttcttcttctcatcggcc

SEQ ID NO: 33 - RNA, 151 nt, synthetic construct
  misc_feature 1..151: note = synthesized sequence
  source 1..151: mol_type = other RNA
gccctggatcatgaagtccttgattacacgatggaatttgctgtttttgtagccaaatcctttctctcctgtagccaaggccacaaaattatccactgtttttggaacagtctttccgaagagaccaaagatcacccggcctacatcttca

SEQ ID NO: 34 - RNA, 72 nt, synthetic construct
  misc_feature 1..72: note = synthesized sequence
  source 1..72: mol_type = other RNA
gcgcaagttaggttttgtcaagaaagggtgtaacgcaaccaagtcatagtccgcctagaagcatttgcggtg

SEQ ID NO: 35 - RNA, 131 nt, synthetic construct
  misc_feature 1..131: note = synthesized sequence
  source 1..131: mol_type = other RNA
gccatgccaatctcatcttgttttctgcgcaagttaggttttgtcaagaaagggtgtaacgcaaccaagtcatagtccgcctagaagcatttgcggtggacgatggaggggccggactcgtcatactcctg

SEQ ID NO: 36 - RNA, 70 nt, synthetic construct
  misc_feature 1..70: note = synthesized sequence
  source 1..70: mol_type = other RNA
ggacttcctgtaacaacgcatctcatatttggaatgaccattaaaaaaacaacaatgtgcaatcaaagtc

SEQ ID NO: 37 - RNA, 71 nt, synthetic construct
  misc_feature 1..71: note = synthesized sequence
  source 1..71: mol_type = other RNA
caaggtgcggctccggcccctcccctcttcaaggggtccacatggcaactgtgaggaggggagattcagtg

SEQ ID NO: 38 - RNA, 91 nt, synthetic construct
  misc_feature 1..91: note = synthesized sequence
  source 1..91: mol_type = other RNA
tagctgtatcgtcaaggcactcgtgccgacgccaccagctccaaccaccacaaggggagagtcagtcagggtcagcaggcctctctcccgc

SEQ ID NO: 39 - RNA, 91 nt, synthetic construct
  misc_feature 1..91: note = synthesized sequence
  source 1..91: mol_type = other RNA
tagctgtatcgtcaaggcactcttgccgacgccaccagctccaaccaccacaagtgtatagtcagtcattttcagcaggcctctctcccgc

SEQ ID NO: 40 - RNA, 91 nt, synthetic construct
  misc_feature 1..91: note = synthesized sequence
  source 1..91: mol_type = other RNA
tagctggatcgtcaaggcactcgtgccgacgccaccagctccaaccaccacaaggggagaggcagtcagggtcagcaggcctctctcccgc

SEQ ID NO: 41 - RNA, 111 nt, synthetic construct
  misc_feature 1..111: note = synthesized sequence
  source 1..111: mol_type = other RNA
gattctgaattagctgtatcgtcaaggcactcttgccgacgccaccagctccaaccaccacaagtgtatagtcagtcattttcagcaggcctctctcccgcacctgggagc

SEQ ID NO: 42 - RNA, 111 nt, synthetic construct
  misc_feature 1..111: note = synthesized sequence
  source 1..111: mol_type = other RNA
gattctgaattagctgtatcgtcaaggcactcgtgccgacgccaccagctccaaccaccacaagtggagagtcagtcattttcagcaggcctctctcccgcacctgggagc

SEQ ID NO: 43 - RNA, 111 nt, synthetic construct
  misc_feature 1..111: note = synthesized sequence
  source 1..111: mol_type = other RNA
gattctgaattagctgtatcgtcaaggcactcgtgccgacgccaccagctccaaccaccacaaggggagagtcagtcagggtcagcaggcctctctcccgcacctgggagc

SEQ ID NO: 44 - RNA, 111 nt, synthetic construct
  misc_feature 1..111: note = synthesized sequence
  source 1..111: mol_type = other RNA
gctccccggtgcgggagagaggcctgctgaccctgactgcctctccccttgtggtggttggagctggtggcgtcggcacgagtgccttgacgatccagctaattcagaatc

SEQ ID NO: 45 - DNA, 71 bp, synthetic construct
  misc_feature 1..71: note = synthesized sequence
  source 1..71: mol_type = other DNA
tctcagtccaatgtatggtccgagcacaagctctaatcaaagtccgcgggtgtagaccggttgccatagga

SEQ ID NO: 46 - RNA, 31 nt, synthetic construct
  misc_feature 1..31: note = synthesized sequence
  source 1..31: mol_type = other RNA
ggaccaccccaaaaatgaaggggactaaaac

SEQ ID NO: 47 - RNA, 70 nt, synthetic construct; identical to SEQ ID NO: 7
  misc_feature 1..70: note = synthesized sequence
  source 1..70: mol_type = other RNA

SEQ ID NO: 48 - RNA, 14 nt, synthetic construct
  misc_feature 1..14: note = synthesized sequence
  source 1..14: mol_type = other RNA
gcagagcctccagc

SEQ ID NO: 49 - RNA, 21 nt, synthetic construct
  misc_feature 1..21: note = synthesized sequence
  source 1..21: mol_type = other RNA
ctcactggcagagcctccagc

SEQ ID NO: 50 - RNA, 27 nt, synthetic construct
  misc_feature 1..27: note = synthesized sequence
  source 1..27: mol_type = other RNA
cccttgctcactggcagagcctccagc

SEQ ID NO: 51 - RNA, 33 nt, synthetic construct
  misc_feature 1..33: note = synthesized sequence
  source 1..33: mol_type = other RNA
ctctcgcccttgctcactggcagagcctccagc

SEQ ID NO: 52 - RNA, 38 nt, synthetic construct
  misc_feature 1..38: note = synthesized sequence
  source 1..38: mol_type = other RNA
ctctcgcccttgctcactggcagagcctccagcatcgc

SEQ ID NO: 53 - RNA, 45 nt, synthetic construct
  misc_feature 1..45: note = synthesized sequence
  source 1..45: mol_type = other RNA
tgaacagctctcgcccttgctcactggcagagcctccagcatcgc

SEQ ID NO: 54 - RNA, 70 nt, synthetic construct; identical to SEQ ID NO: 8
  misc_feature 1..70: note = synthesized sequence
  source 1..70: mol_type = other RNA

SEQ ID NO: 55 - RNA, 70 nt, synthetic construct; identical to SEQ ID NO: 7
  misc_feature 1..70: note = synthesized sequence
  source 1..70: mol_type = other RNA

SEQ ID NO: 56 - RNA, 70 nt, synthetic construct; identical to SEQ ID NO: 8
  misc_feature 1..70: note = synthesized sequence
  source 1..70: mol_type = other RNA

SEQ ID NO: 57 - RNA, 71 nt, synthetic construct
  misc_feature 1..71: note = synthesized sequence
  source 1..71: mol_type = other RNA
tctcagtccaatgtatggtccgagcacaagctctaatcaaagtccgcgggtgtagaccggttgccatagga

SEQ ID NO: 58 - RNA, 71 nt, synthetic construct
  misc_feature 1..71: note = synthesized sequence
  source 1..71: mol_type = other RNA
acagctcctcgcccttgctcactggcagagccctccagcatcgcgagcaggcgctgcctcctccgccgctg

SEQ ID NO: 59 - RNA, 71 nt, synthetic construct
  misc_feature 1..71: note = synthesized sequence
  source 1..71: mol_type = other RNA
acagctcctcgcccttgctcactggcagagccctcaagcatcgcgagcaggcgctgcctcctccgccgctg

SEQ ID NO: 60 - RNA, 71 nt, synthetic construct
  misc_feature 1..71: note = synthesized sequence
  source 1..71: mol_type = other RNA
acagctcctcgcccttgctcactggcagagccctctagcatcgcgagcaggcgctgcctcctccgccgctg

SEQ ID NO: 61 - RNA, 71 nt, synthetic construct
  misc_feature 1..71: note = synthesized sequence
  source 1..71: mol_type = other RNA
acagctcctcgcccttgctcactggcagagccctcgagcatcgcgagcaggcgctgcctcctccgccgctg

SEQ ID NO: 62 - RNA, 71 nt, synthetic construct
  misc_feature 1..71: note = synthesized sequence
  source 1..71: mol_type = other RNA
acagctcctcgcccttgctcactggcagagccctgcagcatcgcgagcaggcgctgcctcctccgccgctg

SEQ ID NO: 63 - RNA, 71 nt, synthetic construct
  misc_feature 1..71: note = synthesized sequence
  source 1..71: mol_type = other RNA
acagctcctcgcccttgctcactggcagagcccttcagcatcgcgagcaggcgctgcctcctccgccgctg

SEQ ID NO: 64 - RNA, 71 nt, synthetic construct
  misc_feature 1..71: note = synthesized sequence
  source 1..71: mol_type = other RNA
acagctcctcgcccttgctcactggcagagccctacagcatcgcgagcaggcgctgcctcctccgccgctg

SEQ ID NO: 65 - RNA, 71 nt, synthetic construct
  misc_feature 1..71: note = synthesized sequence
  source 1..71: mol_type = other RNA
acagctcctcgcccttgctcactggcagagccctcctgcatcgcgagcaggcgctgcctcctccgccgctg

SEQ ID NO: 66 - RNA, 71 nt, synthetic construct
  misc_feature 1..71: note = synthesized sequence
  source 1..71: mol_type = other RNA
acagctcctcgcccttgctcactggcagagccctgctgcatcgcgagcaggcgctgcctcctccgccgctg

SEQ ID NO: 67 - RNA, 71 nt, synthetic construct
  misc_feature 1..71: note = synthesized sequence
  source 1..71: mol_type = other RNA
acagctcctcgcccttgctcactggcagagcccttctgcatcgcgagcaggcgctgcctcctccgccgctg

SEQ ID NO: 68 - RNA, 71 nt, synthetic construct
  misc_feature 1..71: note = synthesized sequence
  source 1..71: mol_type = other RNA
acagctcctcgcccttgctcactggcagagccctactgcatcgcgagcaggcgctgcctcctccgccgctg

SEQ ID NO: 69 - RNA, 71 nt, synthetic construct
  misc_feature 1..71: note = synthesized sequence
  source 1..71: mol_type = other RNA
acagctcctcgcccttgctcactggcagagccctcccgcatcgcgagcaggcgctgcctcctccgccgctg

SEQ ID NO: 70 - RNA, 71 nt, synthetic construct
  misc_feature 1..71: note = synthesized sequence
  source 1..71: mol_type = other RNA
acagctcctcgcccttgctcactggcagagccctgccgcatcgcgagcaggcgctgcctcctccgccgctg

SEQ ID NO: 71 - RNA, 71 nt, synthetic construct
  misc_feature 1..71: note = synthesized sequence
  source 1..71: mol_type = other RNA
acagctcctcgcccttgctcactggcagagcccttccgcatcgcgagcaggcgctgcctcctccgccgctg

SEQ ID NO: 72 - RNA, 71 nt, synthetic construct
  misc_feature 1..71: note = synthesized sequence
  source 1..71: mol_type = other RNA
acagctcctcgcccttgctcactggcagagccctaccgcatcgcgagcaggcgctgcctcctccgccgctg

SEQ ID NO: 73 - RNA, 71 nt, synthetic construct
  misc_feature 1..71: note = synthesized sequence
  source 1..71: mol_type = other RNA
acagctcctcgcccttgctcactggcagagccctccggcatcgcgagcaggcgctgcctcctccgccgctg

SEQ ID NO: 74 - RNA, 71 nt, synthetic construct; identical to SEQ ID NO: 66
  misc_feature 1..71: note = synthesized sequence
  source 1..71: mol_type = other RNA

SEQ ID NO: 75 - RNA, 71 nt, synthetic construct
  misc_feature 1..71: note = synthesized sequence
  source 1..71: mol_type = other RNA
acagctcctcgcccttgctcactggcagagcccttcggcatcgcgagcaggcgctgcctcctccgccgctg

SEQ ID NO: 76 - RNA, 71 nt, synthetic construct
  misc_feature 1..71: note = synthesized sequence
  source 1..71: mol_type = other RNA
acagctcctcgcccttgctcactggcagagccctacggcatcgcgagcaggcgctgcctcctccgccgctg

SEQ ID NO: 77 - RNA, 31 nt, synthetic construct
  misc_feature 1..31: note = synthesized sequence
  source 1..31: mol_type = other RNA
actggcagagccctccagcatcgcgagcagg

SEQ ID NO: 78 - RNA, 51 nt, synthetic construct
  misc_feature 1..51: note = synthesized sequence
  source 1..51: mol_type = other RNA
gcccttgctcactggcagagccctccagcatcgcgagcaggcgctgcctcc

SEQ ID NO: 79 - RNA, 71 nt, synthetic construct; identical to SEQ ID NO: 58
  misc_feature 1..71: note = synthesized sequence
  source 1..71: mol_type = other RNA

SEQ ID NO: 80 - RNA, 91 nt, synthetic construct
  misc_feature 1..91: note = synthesized sequence
  source 1..91: mol_type = other RNA
accccggtgaacagctcctcgcccttgctcactggcagagccctccagcatcgcgagcaggcgctgcctcctccgccgctgcctcctccgc

SEQ ID NO: 81 - RNA, 131 nt, synthetic construct
  misc_feature 1..131: note = synthesized sequence
  source 1..131: mol_type = other RNA
gctcgaccaggatgggcaccaccccggtgaacagctcctcgcccttgctcactggcagagccctccagcatcgcgagcaggcgctgcctcctccgccgctgcctcctccgccgctgcctcctccgccctgc

SEQ ID NO: 82 - RNA, 151 nt, synthetic construct
  misc_feature 1..151: note = synthesized sequence
  source 1..151: mol_type = other RNA
tcgccgtccagctcgaccaggatgggcaccaccccggtgaacagctcctcgcccttgctcactggcagagccctccagcatcgcgagcaggcgctgcctcctccgccgctgcctcctccgccgctgcctcctccgccctgcagcttgtaca

SEQ ID NO: 83 - RNA, 171 nt, synthetic construct
  misc_feature 1..171: note = synthesized sequence
  source 1..171: mol_type = other RNA
gccgtttacgtcgccgtccagctcgaccaggatgggcaccaccccggtgaacagctcctcgcccttgctcactggcagagccctccagcatcgcgagcaggcgctgcctcctccgccgctgcctcctccgccgctgcctcctccgccctgcagcttgtacagctcgtccat

SEQ ID NO: 84 - RNA, 191 nt, synthetic construct
  misc_feature 1..191: note = synthesized sequence
  source 1..191: mol_type = other RNA
tgaacttgtggccgtttacgtcgccgtccagctcgaccaggatgggcaccaccccggtgaacagctcctcgcccttgctcactggcagagccctccagcatcgcgagcaggcgctgcctcctccgccgctgcctcctccgccgctgcctcctccgccctgcagcttgtacagctcgtccatgccgccggtg

SEQ ID NO: 85 - RNA, 211 nt, synthetic construct
  misc_feature 1..211: note = synthesized sequence
  source 1..211: mol_type = other RNA
ccggacacgctgaacttgtggccgtttacgtcgccgtccagctcgaccaggatgggcaccaccccggtgaacagctcctcgcccttgctcactggcagagccctccagcatcgcgagcaggcgctgcctcctccgccgctgcctcctccgccgctgcctcctccgccctgcagcttgtacagctcgtccatgccgccggtggagtggcggc

SEQ ID NO: 86 - RNA, 31 nt, synthetic construct
  misc_feature 1..31: note = synthesized sequence
  source 1..31: mol_type = other RNA
gcgaccggggatctccacagattcttccggc

SEQ ID NO: 87 - RNA, 51 nt, synthetic construct
  misc_feature 1..51: note = synthesized sequence
  source 1..51: mol_type = other RNA
gctcacggtggcgaccggggatctccacagattcttccggcgtgtatacct

SEQ ID NO: 88 - RNA, 71 nt, synthetic construct
  misc_feature 1..71: note = synthesized sequence
  source 1..71: mol_type = other RNA
cctcgcccttgctcacggtggcgaccggggatctccacagattcttccggcgtgtataccttctgctgcct

SEQ ID NO: 89 - RNA, 91 nt, synthetic construct
  misc_feature 1..91: note = synthesized sequence
  source 1..91: mol_type = other RNA
gtgaacagctcctcgcccttgctcacggtggcgaccggggatctccacagattcttccggcgtgtataccttctgctgcctcctccgccgc

SEQ ID NO: 90 - RNA, 111 nt, synthetic construct
  misc_feature 1..111: note = synthesized sequence
  source 1..111: mol_type = other RNA
caccaccccggtgaacagctcctcgcccttgctcacggtggcgaccggggatctccacagattcttccggcgtgtataccttctgctgcctcctccgccgctgcctcctcc

SEQ ID NO: 91 - RNA, 131 nt, synthetic construct
  misc_feature 1..131: note = synthesized sequence
  source 1..131: mol_type = other RNA
ccaggatgggcaccaccccggtgaacagctcctcgcccttgctcacggtggcgaccggggatctccacagattcttccggcgtgtataccttctgctgcctcctccgccgctgcctcctccgccgctgcct

SEQ ID NO: 92 - RNA, 151 nt, synthetic construct
  misc_feature 1..151: note = synthesized sequence
  source 1..151: mol_type = other RNA
tccagctcgaccaggatgggcaccaccccggtgaacagctcctcgcccttgctcacggtggcgaccggggatctccacagattcttccggcgtgtataccttctgctgcctcctccgccgctgcctcctccgccgctgcctcctccgccct

SEQ ID NO: 93 - RNA, 171 nt, synthetic construct
  misc_feature 1..171: note = synthesized sequence
  source 1..171: mol_type = other RNA
cggcgacgtatccagctcgaccaggatgggcaccaccccggtgaacagctcctcgcccttgctcacggtggcgaccggggatctccacagattcttccggcgtgtataccttctgctgcctcctccgccgctgcctcctccgccgctgcctcctccgccctgcagcttgta

SEQ ID NO: 94 - RNA, 191 nt, synthetic construct
  misc_feature 1..191: note = synthesized sequence
  source 1..191: mol_type = other RNA
tgtggccgtttacgtcgccgtccagctcgaccaggatgggcaccaccccggtgaacagctcctcgcccttgctcacggtggcgaccggggatctccacagattcttccggcgtgtataccttctgctgcctcctccgccgctgcctcctccgccgctgcctcctccgccctgcagcttgtacagctcgtcc

SEQ ID NO: 95 - RNA, 211 nt, synthetic construct
  misc_feature 1..211: note = synthesized sequence
  source 1..211: mol_type = other RNA
acgctgaacttgtggccgtttacgtcgccgtccagctcgaccaggatgggcaccaccccggtgaacagctcctcgcccttgctcacggtggcgaccggggatctccacagattcttccggcgtgtataccttctgctgcctcctccgccgctgcctcctccgccgctgcctcctccgccctgcagcttgtacagctcgtccatgccgccgg

SEQ ID NO: 96 - RNA, 71 nt, synthetic construct
  misc_feature 1..71: note = synthesized sequence
  source 1..71: mol_type = other RNA
cagcatcgcgagcaggcgctgcctcctccgccgctgcctcctccgccgctgcctcctccgccctgcagctt

SEQ ID NO: 97 - RNA, 71 nt, synthetic construct
  misc_feature 1..71: note = synthesized sequence
  source 1..71: mol_type = other RNA
ccctccagcatcgcgagcaggcgctgcctcctccgccgctgcctcctccgccgctgcctcctccgccctgc

SEQ ID NO: 98 - RNA, 71 nt, synthetic construct
  misc_feature 1..71: note = synthesized sequence
  source 1..71: mol_type = other RNA
cagagccctccagcatcgcgagcaggcgctgcctcctccgccgctgcctcctccgccgctgcctcctccgc

SEQ ID NO: 99 - RNA, 72 nt, synthetic construct
  misc_feature 1..72: note = synthesized sequence
  source 1..72: mol_type = other RNA
actggcagagccctcccagcatcgcgagcaggcgctgcctcctccgccgctgcctcctccgccgctgcctcc

SEQ ID NO: 100 - RNA, 71 nt, synthetic construct
  misc_feature 1..71: note = synthesized sequence
  source 1..71: mol_type = other RNA
tgctcactggcagagccctccagcatcgcgagcaggcgctgcctcctccgccgctgcctcctccgccgctg

SEQ ID NO: 101 - RNA, 71 nt, synthetic construct
  misc_feature 1..71: note = synthesized sequence
  source 1..71: mol_type = other RNA
gcccttgctcactggcagagccctccagcatcgcgagcaggcgctgcctcctccgccgctgcctcctccgc

SEQ ID NO: 102 - RNA, 71 nt, synthetic construct
  misc_feature 1..71: note = synthesized sequence
  source 1..71: mol_type = other RNA
tcctcgcccttgctcactggcagagccctccagcatcgcgagcaggcgctgcctcctccgccgctgcctcc

SEQ ID NO: 103 - RNA, 71 nt, synthetic construct
  misc_feature 1..71: note = synthesized sequence
  source 1..71: mol_type = other RNA
ggtgaacagctcctcgcccttgctcactggcagagccctccagcatcgcgagcaggcgctgcctcctccgc

SEQ ID NO: 104 - RNA, 71 nt, synthetic construct
  misc_feature 1..71: note = synthesized sequence
  source 1..71: mol_type = other RNA
accccggtgaacagctcctcgcccttgctcactggcagagccctccagcatcgcgagcaggcgctgcctcc

SEQ ID NO: 105 - RNA, 71 nt, synthetic construct
  misc_feature 1..71: note = synthesized sequence
  source 1..71: mol_type = other RNA
gcaccaccccggtgaacagctcctcgcccttgctcactggcagagccctccagcatcgcgagcaggcgctg

SEQ ID NO: 106 - RNA, 71 nt, synthetic construct
  misc_feature 1..71: note = synthesized sequence
  source 1..71: mol_type = other RNA
gatgggcaccaccccggtgaacagctcctcgcccttgctcactggcagagccctccagcatcgcgagcagg

SEQ ID NO: 107 - RNA, 71 nt, synthetic construct
  misc_feature 1..71: note = synthesized sequence
  source 1..71: mol_type = other RNA
accaggatgggcaccaccccggtgaacagctcctcgcccttgctcactggcagagccctccagcatcgcga

SEQ ID NO: 108 - RNA, 71 nt, synthetic construct
  misc_feature 1..71: note = synthesized sequence
  source 1..71: mol_type = other RNA
gctcgaccaggatgggcaccaccccggtgaacagctcctcgcccttgctcactggcagagccctccagcat

SEQ ID NO: 109 - RNA, 71 nt, synthetic construct
  misc_feature 1..71: note = synthesized sequence
  source 1..71: mol_type = other RNA
gtccagctcgaccaggatgggcaccaccccggtgaacagctcctcgcccttgctcactggcagagccctcc

SEQ ID NO: 110 - RNA, 71 nt, synthetic construct
  misc_feature 1..71: note = synthesized sequence
  source 1..71: mol_type = other RNA
cacagattcttccggcgtgtataccttctgctgcctcctccgccgctgcctcctccgccgctgcctcctcc

SEQ ID NO: 111 - RNA, 71 nt, synthetic construct
  misc_feature 1..71: note = synthesized sequence
  source 1..71: mol_type = other RNA
atctccacagattcttccggcgtgtataccttctgctgcctcctccgccgctgcctcctccgccgctgcct

SEQ ID NO: 112 - RNA, 71 nt, synthetic construct
  misc_feature 1..71: note = synthesized sequence
  source 1..71: mol_type = other RNA
cggggatctccacagattcttccggcgtgtataccttctgctgcctcctccgccgctgcctcctccgccgc

SEQ ID NO: 113 - RNA, 71 nt, synthetic construct
  misc_feature 1..71: note = synthesized sequence
  source 1..71: mol_type = other RNA
gcgaccggggatctccacagattcttccggcgtgtataccttctgctgcctcctccgccgctgcctcctcc

SEQ ID NO: 114 - RNA, 71 nt, synthetic construct
  misc_feature 1..71: note = synthesized sequence
  source 1..71: mol_type = other RNA
cggtggcgaccggggatctccacagattcttccggcgtgtataccttctgctgcctcctccgccgctgcct

SEQ ID NO: 115 - RNA, 71 nt, synthetic construct
  misc_feature 1..71: note = synthesized sequence
  source 1..71: mol_type = other RNA
gctcacggtggcgaccggggatctccacagattcttccggcgtgtataccttctgctgcctcctccgccgc

SEQ ID NO: 116 - RNA, 71 nt, synthetic construct
  misc_feature 1..71: note = synthesized sequence
  source 1..71: mol_type = other RNA
cccttgctcacggtggcgaccggggatctccacagattcttccggcgtgtataccttctgctgcctcctcc

SEQ ID NO: 117 - RNA, 71 nt, synthetic construct
  misc_feature 1..71: note = synthesized sequence
  source 1..71: mol_type = other RNA
cagctcctcgcccttgctcacggtggcgaccggggatctccacagattcttccggcgtgtataccttctgc

SEQ ID NO: 118 - RNA, 71 nt, synthetic construct
  misc_feature 1..71: note = synthesized sequence
  source 1..71: mol_type = other RNA
gtgaacagctcctcgcccttgctcacggtggcgaccggggatctccacagattcttccggcgtgtatacct

SEQ ID NO: 119 - RNA, 71 nt, synthetic construct
  misc_feature 1..71: note = synthesized sequence
  source 1..71: mol_type = other RNA
ccccggtgaacagctcctcgcccttgctcacggtggcgaccggggatctccacagattcttccggcgtgta

SEQ ID NO: 120 - RNA, 71 nt, synthetic construct
  misc_feature 1..71: note = synthesized sequence
  source 1..71: mol_type = other RNA
caccaccccggtgaacagctcctcgcccttgctcacggtggcgaccggggatctccacagattcttccggc

SEQ ID NO: 121 - RNA, 71 nt, synthetic construct
  misc_feature 1..71: note = synthesized sequence
  source 1..71: mol_type = other RNA
atgggcaccaccccggtgaacagctcctcgcccttgctcacggtggcgaccggggatctccacagattctt

SEQ ID NO: 122 - RNA, 71 nt, synthetic construct
  misc_feature 1..71: note = synthesized sequence
  source 1..71: mol_type = other RNA
ccaggatgggcaccaccccggtgaacagctcctcgcccttgctcacggtggcgaccggggatctccacaga

SEQ ID NO: 123 - RNA, 71 nt, synthetic construct
  misc_feature 1..71: note = synthesized sequence
  source 1..71: mol_type = other RNA
ctcgaccaggatgggcaccaccccggtgaacagctcctcgcccttgctcacggtggcgaccggggatctcc

SEQ ID NO: 124 - RNA, 111 nt, synthetic construct
  misc_feature 1..111: note = synthesized sequence
  source 1..111: mol_type = other RNA
gatgggcaccaccccggtgaacagctcctcgcccttgctcactggcagagccctccagcatcgcgagcaggcgctgcctcctccgccctgcagcttgtacagctcgtccat

SEQ ID NO: 125 - RNA, 111 nt, synthetic construct
  misc_feature 1..111: note = synthesized sequence
  source 1..111: mol_type = other RNA
gatgggcaccaccccggtgaacagctcctcgcccttgctcactggcagagccctgcagcatcgcgagcaggcgctgcctcctccgccctgcagcttgtacagctcgtccat

SEQ ID NO: 126 - RNA, 111 nt, synthetic construct
  misc_feature 1..111: note = synthesized sequence
  source 1..111: mol_type = other RNA
gatgggcaccaccccggtgaacagctcctcgcccttgctcactggcagagcccttcagcatcgcgagcaggcgctgcctcctccgccctgcagcttgtacagctcgtccat

SEQ ID NO: 127 - RNA, 111 nt, synthetic construct
  misc_feature 1..111: note = synthesized sequence
  source 1..111: mol_type = other RNA
gatgggcaccaccccggtgaacagctcctcgcccttgctcactggcagagccctacagcatcgcgagcaggcgctgcctcctccgccctgcagcttgtacagctcgtccat

SEQ ID NO: 128 - RNA, 111 nt, synthetic construct
  misc_feature 1..111: note = synthesized sequence
  source 1..111: mol_type = other RNA
gatgggcaccaccccggtgaacagctcctcgcccttgctcactggcagagccctccggcatcgcgagcaggcgctgcctcctccgccctgcagcttgtacagctcgtccat

SEQ ID NO: 129 - RNA, 111 nt, synthetic construct
  misc_feature 1..111: note = synthesized sequence
  source 1..111: mol_type = other RNA
gatgggcaccaccccggtgaacagctcctcgcccttgctcactggcagagccctgcggcatcgcgagcaggcgctgcctcctccgccctgcagcttgtacagctcgtccat

SEQ ID NO: 130 - RNA, 111 nt, synthetic construct
  source 1..111: mol_type = other RNA
  misc_feature 1..111: note = synthesized sequence
gatgggcaccaccccggtgaacagctcctcgcccttgctcactggcagagcccttcggcatcgcgagcaggcgctgcctcctccgccctgcagcttgtacagctcgtccat

SEQ ID NO: 131 - RNA, 111 nt, synthetic construct
  misc_feature 1..111: note = synthesized sequence
  source 1..111: mol_type = other RNA
gatgggcaccaccccggtgaacagctcctcgcccttgctcactggcagagccctacggcatcgcgagcaggcgctgcctcctccgccctgcagcttgtacagctcgtccat

SEQ ID NO: 132 - RNA, 111 nt, synthetic construct
  misc_feature 1..111: note = synthesized sequence
  source 1..111: mol_type = other RNA
gatgggcaccaccccggtgaacagctcctcgcccttgctcactggcagagccctcctgcatcgcgagcaggcgctgcctcctccgccctgcagcttgtacagctcgtccat

SEQ ID NO: 133 - RNA, 111 nt, synthetic construct
  misc_feature 1..111: note = synthesized sequence
  source 1..111: mol_type = other RNA
gatgggcaccaccccggtgaacagctcctcgcccttgctcactggcagagccctgctgcatcgcgagcaggcgctgcctcctccgccctgcagcttgtacagctcgtccat

SEQ ID NO: 134 - RNA, 111 nt, synthetic construct
  misc_feature 1..111: note = synthesized sequence
  source 1..111: mol_type = other RNA
gatgggcaccaccccggtgaacagctcctcgcccttgctcactggcagagccctactgcatcgcgagcaggcgctgcctcctccgccctgcagcttgtacagctcgtccat

SEQ ID NO: 135 - RNA, 111 nt, synthetic construct
  misc_feature 1..111: note = synthesized sequence
  source 1..111: mol_type = other RNA
gatgggcaccaccccggtgaacagctcctcgcccttgctcactggcagagcccttctgcatcgcgagcaggcgctgcctcctccgccctgcagcttgtacagctcgtccat

SEQ ID NO: 136 - RNA, 111 nt, synthetic construct
  misc_feature 1..111: note = synthesized sequence
  source 1..111: mol_type = other RNA
gatgggcaccaccccggtgaacagctcctcgcccttgctcactggcagagccctcccgcatcgcgagcaggcgctgcctcctccgccctgcagcttgtacagctcgtccat

SEQ ID NO: 137 - RNA, 111 nt, synthetic construct
  misc_feature 1..111: note = synthesized sequence
  source 1..111: mol_type = other RNA
gatgggcaccaccccggtgaacagctcctcgcccttgctcactggcagagccctgccgcatcgcgagcaggcgctgcctcctccgccctgcagcttgtacagctcgtccat

SEQ ID NO: 138 - RNA, 111 nt, synthetic construct
  misc_feature 1..111: note = synthesized sequence
  source 1..111: mol_type = other RNA
gatgggcaccaccccggtgaacagctcctcgcccttgctcactggcagagcccttccgcatcgcgagcaggcgctgcctcctccgccctgcagcttgtacagctcgtccat

SEQ ID NO: 139 - RNA, 111 nt, synthetic construct
  misc_feature 1..111: note = synthesized sequence
  source 1..111: mol_type = other RNA
gatgggcaccaccccggtgaacagctcctcgcccttgctcactggcagagccctaccgcatcgcgagcaggcgctgcctcctccgccctgcagcttgtacagctcgtccat

SEQ ID NO: 140 - RNA, 111 nt, synthetic construct
  misc_feature 1..111: note = synthesized sequence
  source 1..111: mol_type = other RNA
taccgctacagccacgctgatttcagctatacctgcccggtataaagggacgttcacaccgcgatgttctctgctggggaattgcgcgatattcaggattaaaagaagtgc

SEQ ID NO: 141 - RNA, 151 nt, synthetic construct
  misc_feature 1..151: note = synthesized sequence
  source 1..151: mol_type = other RNA
actacagttgctccgatatttaggctacgtcaataggcactaacttattggcgctggtgaacggacttcctctcgagtaccagaagatgactacaaaactcctttccattgcgagtatcggagtctggctcagtttggccagggaggcact

SEQ ID NO: 142 - RNA, 51 nt, synthetic construct
  misc_feature 1..51: note = synthesized sequence
  source 1..51: mol_type = other RNA
cggaagagggtggggccgcggtggccagggagccggcgccgccacgcgcgg

SEQ ID NO: 143 - RNA, 71 nt, synthetic construct
  misc_feature 1..71: note = synthesized sequence
  source 1..71: mol_type = other RNA
cagctgaggccggaagagggtggggccgcggtggccagggagccggcgccgccacgcgcgggtggggggga

SEQ ID NO: 144 - RNA, 111 nt, synthetic construct
  misc_feature 1..111: note = synthesized sequence
  source 1..111: mol_type = other RNA
ggaggcgaaagcagcccggacagctgaggccggaagagggtggggccgcggtggccagggagccggcgccgccacgcgcgggtgggggggactggggttgctcgcgggctc

SEQ ID NO: 145 - RNA, 151 nt, synthetic construct; identical to SEQ ID NO: 31
  misc_feature 1..151: note = synthesized sequence
  source 1..151: mol_type = other RNA

SEQ ID NO: 146 - RNA, 51 nt, synthetic construct
  misc_feature 1..51: note = synthesized sequence
  source 1..51: mol_type = other RNA
tcttgcctacgccaccagctccaaccaccacaagtttatattcagtcattt

SEQ ID NO: 147 - RNA, 111 nt, synthetic construct
  misc_feature 1..111: note = synthesized sequence
  source 1..111: mol_type = other RNA
gattctgaattagctgtatcgtcaaggcactcttgcctacgccaccagctccaaccaccacaagtttatattcagtcattttcagcaggcctctctcccgcacctgggagc

SEQ ID NO: 148 - RNA, 151 nt, synthetic construct; identical to SEQ ID NO: 28
  misc_feature 1..151: note = synthesized sequence
  source 1..151: mol_type = other RNA

SEQ ID NO: 149 - RNA, 51 nt, synthetic construct
  misc_feature 1..51: note = synthesized sequence
  source 1..51: mol_type = other RNA
tcggcatggtatgaagtacttcgtccaggagctggagggcccggtgtaagt

SEQ ID NO: 150 - RNA, 71 nt, synthetic construct
  misc_feature 1..71: note = synthesized sequence
  source 1..71: mol_type = other RNA
gggtctgcaatcggcatggtatgaagtacttcgtccaggagctggagggcccggtgtaagtgaatttcaat

SEQ ID NO: 151 - RNA, 111 nt, synthetic construct
  misc_feature 1..111: note = synthesized sequence
  source 1..111: mol_type = other RNA
gacctcagtctaaaggttgtgggtctgcaatcggcatggtatgaagtacttcgtccaggagctggagggcccggtgtaagtgaatttcaatccagcaaggtgtttctttga

SEQ ID NO: 152 - RNA, 151 nt, synthetic construct
  misc_feature 1..151: note = synthesized sequence
  source 1..151: mol_type = other RNA
taagggccccaacggtaaaagacctcagtctaaaggttgtgggtctgcaatcggcatggtatgaagtacttcgtccaggagctggagggcccggtgtaagtgaatttcaatccagcaaggtgtttctttgatgctctgtcttgggtaatcc

SEQ ID NO: 153 - RNA, 51 nt, synthetic construct
  misc_feature 1..51: note = synthesized sequence
  source 1..51: mol_type = other RNA
tggggggttcggctgccgacatcagcaattgctctgccaccatctcagccc

SEQ ID NO: 154 - RNA, 71 nt, synthetic construct
  misc_feature 1..71: note = synthesized sequence
  source 1..71: mol_type = other RNA
agcagggccgtggggggttcggctgccgacatcagcaattgctctgccaccatctcagcccatcctccgaa

SEQ ID NO: 155 - RNA, 111 nt, synthetic construct
  misc_feature 1..111: note = synthesized sequence
  source 1..111: mol_type = other RNA
agtagaaggccaagagccacagcagggccgtggggggttcggctgccgacatcagcaattgctctgccaccatctcagcccatcctccgaagtgaatgaacaggaaccagc

SEQ ID NO: 156 - RNA, 151 nt, synthetic construct
  misc_feature 1..151: note = synthesized sequence
  source 1..151: mol_type = other RNA
cctcccatcacgggggccgtagtagaaggccaagagccacagcagggccgtggggggttcggctgccgacatcagcaattgctctgccaccatctcagcccatcctccgaagtgaatgaacaggaaccagctctcaaagggacctccgcag

SEQ ID NO: 157 - DNA, 151 bp, synthetic construct
  misc_feature 1..151: note = synthesized sequence
  source 1..151: mol_type = other DNA
gccaaacaccacatgcttgccatctagccaggctgtcttgactgtcgtgatgaagaactgggagccgttggtgtccttgcctgcgttggccatgctcacccagccaggcccgtagtgcttcagtttgaagttctcatcggggaagcgctca

SEQ ID NO: 158 - DNA, 151 bp, synthetic construct
  misc_feature 1..151: note = synthesized sequence
  source 1..151: mol_type = other DNA
gggagtgggtccgctccaccagatgccagcaccggggccagtgcagctcagagccctgtggcggactacagggcccgcacagacggtcactcaaagaaagatgtccctgtgccctactccttggcgatggcaaagggcttctccacctcga

SEQ ID NO: 159 - DNA, 151 bp, synthetic construct
  misc_feature 1..151: note = synthesized sequence
  source 1..151: mol_type = other DNA
tgcattttgtaaaatagatactagcagattgtcccaagatgtgtacagctcattctcacagcccagcgagggcacctactccacaaatgcgtggccacaggtcatcacctgtcctgtggccctggcgagcctgatccctcacgccgggcac

SEQ ID NO: 160 - DNA, 151 bp, synthetic construct
  misc_feature 1..151: note = synthesized sequence
  source 1..151: mol_type = other DNA
gctcattctcacagcccagcgagggcacttactccacaaatgcgtggccacaggtcatcacctgtcctgtggccccggcgagcctgatccctcacgccgggcacccacacggcctgcgtgccttctagacttgagttcgcagctctttaag

SEQ ID NO: 161 - DNA, 151 bp, synthetic construct
  misc_feature 1..151: note = synthesized sequence
  source 1..151: mol_type = other DNA
tcggccgggccctgggggcggtgggcgctggccaggacgcccaccgtgtggttgctgtccaggacggtcccggcccgcgacacttcggcccagagctgctcctcatccagcagcgccagcagccccatggccgtgagcaccggcttgcgca

SEQ ID NO: 162 - RNA, 111 nt, synthetic construct
  misc_feature 1..111: note = synthesized sequence
  source 1..111: mol_type = other RNA
tgaccagtcttaagatctttcttgacctgcaccataagaacttctccaaaggtaccaaaatactctttcaggtcctgttcggttgttttccatgggagacccaacactatt

SEQ ID NO: 163 - RNA, 111 nt, synthetic construct
  misc_feature 1..111: note = synthesized sequence
  source 1..111: mol_type = other RNA
gatgggcaccaccccggtgaacagctcctcgcccttgctcactggcagagccctcgagcatcgcgagcaggcgctgcctcctccgccctgcagcttgtacagctcgtccat

SEQ ID NO: 164 - RNA, 111 nt, synthetic construct
  misc_feature 1..111: note = synthesized sequence
  source 1..111: mol_type = other RNA
gatgggcaccaccccggtgaacagctcctcgcccttgctcactggcagagccctggagcatcgcgagcaggcgctgcctcctccgccctgcagcttgtacagctcgtccat

SEQ ID NO: 165 - RNA, 111 nt, synthetic construct
  misc_feature 1..111: note = synthesized sequence
  source 1..111: mol_type = other RNA
gatgggcaccaccccggtgaacagctcctcgcccttgctcactggcagagcccttgagcatcgcgagcaggcgctgcctcctccgccctgcagcttgtacagctcgtccat

SEQ ID NO: 166 - RNA, 111 nt, synthetic construct
  misc_feature 1..111: note = synthesized sequence
  source 1..111: mol_type = other RNA
gatgggcaccaccccggtgaacagctcctcgcccttgctcactggcagagccctagagcatcgcgagcaggcgctgcctcctccgccctgcagcttgtacagctcgtccat

SEQ ID NO: 167 - RNA, 111 nt, synthetic construct
  misc_feature 1..111: note = synthesized sequence
  source 1..111: mol_type = other RNA
gatgggcaccaccccggtgaacagctcctcgcccttgctcactggcagagccctcgggcatcgcgagcaggcgctgcctcctccgccctgcagcttgtacagctcgtccat

SEQ ID NO: 168 - RNA, 111 nt, synthetic construct
  misc_feature 1..111: note = synthesized sequence
  source 1..111: mol_type = other RNA
gatgggcaccaccccggtgaacagctcctcgcccttgctcactggcagagccctggggcatcgcgagcaggcgctgcctcctccgccctgcagcttgtacagctcgtccat

SEQ ID NO: 169 - RNA, 111 nt, synthetic construct
  misc_feature 1..111: note = synthesized sequence
  source 1..111: mol_type = other RNA
gatgggcaccaccccggtgaacagctcctcgcccttgctcactggcagagcccttgggcatcgcgagcaggcgctgcctcctccgccctgcagcttgtacagctcgtccat

SEQ ID NO: 170 - RNA, 111 nt, synthetic construct
  misc_feature 1..111: note = synthesized sequence
  source 1..111: mol_type = other RNA
gatgggcaccaccccggtgaacagctcctcgcccttgctcactggcagagccctagggcatcgcgagcaggcgctgcctcctccgccctgcagcttgtacagctcgtccat

SEQ ID NO: 171 - RNA, 111 nt, synthetic construct
  misc_feature 1..111: note = synthesized sequence
  source 1..111: mol_type = other RNA
gatgggcaccaccccggtgaacagctcctcgcccttgctcactggcagagccctcgtgcatcgcgagcaggcgctgcctcctccgccctgcagcttgtacagctcgtccat

SEQ ID NO: 172 - RNA, 111 nt, synthetic construct
  misc_feature 1..111: note = synthesized sequence
  source 1..111: mol_type = other RNA
gatgggcaccaccccggtgaacagctcctcgcccttgctcactggcagagccctggtgcatcgcgagcaggcgctgcctcctccgccctgcagcttgtacagctcgtccat

SEQ ID NO: 173 - RNA, 111 nt, synthetic construct
  misc_feature 1..111: note = synthesized sequence
  source 1..111: mol_type = other RNA
gatgggcaccaccccggtgaacagctcctcgcccttgctcactggcagagccctagtgcatcgcgagcaggcgctgcctcctccgccctgcagcttgtacagctcgtccat

SEQ ID NO: 174 - RNA, 111 nt, synthetic construct
  misc_feature 1..111: note = synthesized sequence
  source 1..111: mol_type = other RNA
gatgggcaccaccccggtgaacagctcctcgcccttgctcactggcagagcccttgtgcatcgcgagcaggcgctgcctcctccgccctgcagcttgtacagctcgtccat

SEQ ID NO: 175 - RNA, 111 nt, synthetic construct
  misc_feature 1..111: note = synthesized sequence
  source 1..111: mol_type = other RNA
gatgggcaccaccccggtgaacagctcctcgcccttgctcactggcagagccctcgcgcatcgcgagcaggcgctgcctcctccgccctgcagcttgtacagctcgtccat

SEQ ID NO: 176 - RNA, 111 nt, synthetic construct
  misc_feature 1..111: note = synthesized sequence
  source 1..111: mol_type = other RNA
gatgggcaccaccccggtgaacagctcctcgcccttgctcactggcagagccctggcgcatcgcgagcaggcgctgcctcctccgccctgcagcttgtacagctcgtccat

SEQ ID NO: 177 - RNA, 111 nt, synthetic construct
  misc_feature 1..111: note = synthesized sequence
  source 1..111: mol_type = other RNA
gatgggcaccaccccggtgaacagctcctcgcccttgctcactggcagagcccttgcgcatcgcgagcaggcgctgcctcctccgccctgcagcttgtacagctcgtccat

SEQ ID NO: 178 - RNA, 111 nt, synthetic construct
  misc_feature 1..111: note = synthesized sequence
  source 1..111: mol_type = other RNA
gatgggcaccaccccggtgaacagctcctcgcccttgctcactggcagagccctagcgcatcgcgagcaggcgctgcctcctccgccctgcagcttgtacagctcgtccat

SEQ ID NO: 179 - RNA, 111 nt, synthetic construct; identical to SEQ ID NO: 163
  misc_feature 1..111: note = synthesized sequence
  source 1..111: mol_type = other RNA

SEQ ID NO: 180 - RNA, 111 nt, synthetic construct; identical to SEQ ID NO: 164
  misc_feature 1..111: note = synthesized sequence
  source 1..111: mol_type = other RNA

SEQ ID NO: 181 - RNA, 111 nt, synthetic construct; identical to SEQ ID NO: 165
  misc_feature 1..111: note = synthesized sequence
  source 1..111: mol_type = other RNA

SEQ ID NO: 182 - RNA, 111 nt, synthetic construct; identical to SEQ ID NO: 166
  misc_feature 1..111: note = synthesized sequence
  source 1..111: mol_type = other RNA

SEQ ID NO: 183 - RNA, 111 nt, synthetic construct; identical to SEQ ID NO: 171
  misc_feature 1..111: note = synthesized sequence
  source 1..111: mol_type = other RNA

SEQ ID NO: 184 - RNA, 111 nt, synthetic construct; identical to SEQ ID NO: 167
  misc_feature 1..111: note = synthesized sequence
  source 1..111: mol_type = other RNA

SEQ ID NO: 185 - RNA, 111 nt, synthetic construct; identical to SEQ ID NO: 175
  misc_feature 1..111: note = synthesized sequence
  source 1..111: mol_type = other RNA

SEQ ID NO: 186 - RNA, 111 nt, synthetic construct; identical to SEQ ID NO: 171
  misc_feature 1..111: note = synthesized sequence
  source 1..111: mol_type = other RNA

SEQ ID NO: 187 - RNA, 111 nt, synthetic construct; identical to SEQ ID NO: 172
  misc_feature 1..111: note = synthesized sequence
  source 1..111: mol_type = other RNA

SEQ ID NO: 188 - RNA, 111 nt, synthetic construct; identical to SEQ ID NO: 174
  misc_feature 1..111: note = synthesized sequence
  source 1..111: mol_type = other RNA

SEQ ID NO: 189 - RNA, 111 nt, synthetic construct; identical to SEQ ID NO: 173
  misc_feature 1..111: note = synthesized sequence
  source 1..111: mol_type = other RNA

SEQ ID NO: 190 - RNA, 111 nt, synthetic construct; identical to SEQ ID NO: 163
  misc_feature 1..111: note = synthesized sequence
  source 1..111: mol_type = other RNA

SEQ ID NO: 191 - RNA, 111 nt, synthetic construct; identical to SEQ ID NO: 175
  misc_feature 1..111: note = synthesized sequence
  source 1..111: mol_type = other RNA

SEQ ID NO: 192 - RNA, 111 nt, synthetic construct; identical to SEQ ID NO: 167
  misc_feature 1..111: note = synthesized sequence
  source 1..111: mol_type = other RNA

SEQ ID NO: 193 - RNA, 111 nt, synthetic construct; identical to SEQ ID NO: 42
  misc_feature 1..111: note = synthesized sequence
  source 1..111: mol_type = other RNA

SEQ ID NO: 194 - RNA, 111 nt, synthetic construct
  misc_feature 1..111: note = synthesized sequence
  source 1..111: mol_type = other RNA
gattctgaattagctggatcgtcaaggcactcgggccgacgccaccagctccaaccaccacaagtggagagtcagtcattttcagcaggcctctctcccgcaccggggagc

SEQ ID NO: 195 - RNA, 111 nt, synthetic construct
  misc_feature 1..111: note = synthesized sequence
  source 1..111: mol_type = other RNA
gggagcagcctctggcattctgggagcttcatctggacctgggtcttcagtgaaccattgttcaatatcgtccggggacagcatcaaatcatccattgcttgggacggcaa

SEQ ID NO: 196 - RNA, 111 nt, synthetic construct
  misc_feature 1..111: note = synthesized sequence
  source 1..111: mol_type = other RNA
gggagcagcctctggcattctgggagcttcatctggacctgggtcttcagtgaaccattgttcaagatcgtccggggacagcatcaaatcatccattgcttgggacggcaa

SEQ ID NO: 197 - RNA, 111 nt, synthetic construct
  misc_feature 1..111: note = synthesized sequence
  source 1..111: mol_type = other RNA
gggagcagcctctggcagtcggggagcttcatctggacctgggtcttcagtgaaccattgttcaagatcgtccggggacagcatcaaatcatccagtgcttgggacggcaa

SEQ ID NO: 198 - RNA, 111 nt, synthetic construct
  misc_feature 1..111: note = synthesized sequence
  source 1..111: mol_type = other RNA
catattacagaataccttgatagcatccaatttgcatccttggttagggtcaacccagtattctccactcttgagttcaggatggcagaatttcaggtctctgcagtttct

SEQ ID NO: 199 - RNA, 111 nt, synthetic construct
  misc_feature 1..111: note = synthesized sequence
  source 1..111: mol_type = other RNA
gtgaagataagccagtcctctagtaacagaatgagcaagacggcaagagcttacccagtcacttgtgtggagacttaaatacttgcataaagatccattgggatagtactc

SEQ ID NO: 200 - RNA, 111 nt, synthetic construct
  misc_feature 1..111: note = synthesized sequence
  source 1..111: mol_type = other RNA
gtgaacgtcaaactgtcggaccaatatggcagaatcttctctcatctcaactttccatatccgtatcatggaatcatagcatcctgtaactactagctctcttacagctgg

SEQ ID NO: 201 - RNA, 111 nt, synthetic construct
  misc_feature 1..111: note = synthesized sequence
  source 1..111: mol_type = other RNA
gccaatgatctcgtgagttatctcagcagtgtgagccatcagggtgatgacatcccaggcgatcgtgtggcctccaggagcccagagcaggaagttgaggagaaggtgcct

SEQ ID NO: 202 - RNA, 111 nt, synthetic construct
  misc_feature 1..111: note = synthesized sequence
  source 1..111: mol_type = other RNA
caagacggtgaaccactccatggtcttcttgtcggctttctgcactgtgtacccccagagctccgtgttgccgacatcctggggtggcttccactccagagccacattaag

SEQ ID NO: 203 - RNA, 111 nt, synthetic construct
  misc_feature 1..111: note = synthesized sequence
  source 1..111: mol_type = other RNA
aggattctcttttgaagtattgctcccccagtggattgggtggctccattcactccaatgctgagcacttccacagagtgggttaaagcggctccgaacacgaaacgtgta

SEQ ID NO: 204 - RNA, 111 nt, synthetic construct
  misc_feature 1..111: note = synthesized sequence
  source 1..111: mol_type = other RNA
gacgcccaccgtgtggttgctgtccaggacggtcccggcctgcgacacttcggcccagagctgctcctcatccagcagcgccagcagccccatggccgtgagcaccggctt

SEQ ID NO: 205 - RNA, 111 nt, synthetic construct
  misc_feature 1..111: note = synthesized sequence
  source 1..111: mol_type = other RNA
gacgcccaccgtgtggttgctgtccaggacggtcccggcctgcgacacttcggcccagagctgctcctcatctgcggggcgggggggggccgtcgccgcgtggggtcgttg

SEQ ID NO: 206 - DNA, 31 bp, synthetic construct
  misc_feature 1..31: note = synthesized sequence
  source 1..31: mol_type = other DNA
tataactagtatggtgagcaagggcgaggag

SEQ ID NO: 207 - DNA, 41 bp, synthetic construct
  misc_feature 1..41: note = synthesized sequence
  source 1..41: mol_type = other DNA
tatacgtctcatctacagattcttccggcgtgtataccttc

SEQ ID NO: 208 - DNA, 53 bp, synthetic construct
  misc_feature 1..53: note = synthesized sequence
  source 1..53: mol_type = other DNA
tatacgtctcatagagatccccggtcgccaccgtgagcaagggcgaggagctg

SEQ ID NO: 209 - DNA, 36 bp, synthetic construct
  misc_feature 1..36: note = synthesized sequence
  source 1..36: mol_type = other DNA
tataggcgcgccttacttgtacagctcgtccatgcc

SEQ ID NO: 210 - DNA, 94 bp, synthetic construct
  misc_feature 1..94: note = synthesized sequence
  source 1..94: mol_type = other DNA
tatacgtctcaaggcgctgcctcctccgccgctgcctcctccgccgctgcctcctccgccctgcagcttgtacagctcgtccatgccgccggtg

SEQ ID NO: 211 - DNA, 62 bp, synthetic construct
  misc_feature 1..62: note = synthesized sequence
  source 1..62: mol_type = other DNA
tatacgtctcagcctgctcgcgatgctagagggctctgccagtgagcaagggcgaggagctg

SEQ ID NO: 212 - DNA, 70 bp, synthetic construct
  misc_feature 1..70: note = synthesized sequence
  source 1..70: mol_type = other DNA
tataactagtatggtggattacaaggatgacgacgataagatgaaagtgacgaaggtaggaggcatttcg

SEQ ID NO: 213 - DNA, 60 bp, synthetic construct
  misc_feature 1..60: note = synthesized sequence
  source 1..60: mol_type = other DNA
atatggcgcgccgttttcagactttttctcttccattttgtattcaaacataatcttcac

SEQ ID NO: 214 - DNA, 69 bp, synthetic construct
  misc_feature 1..69: note = synthesized sequence
  source 1..69: mol_type = other DNA
tataggcgcgccaggcggaggaggcagcggcggaggaggcagcctcctcctctcaaggtccccagaagc

SEQ ID NO: 215 - DNA, 64 bp, synthetic construct
  misc_feature 1..64: note = synthesized sequence
  source 1..64: mol_type = other DNA
tatacctgcaggctacaccttgcgttttttcttgggtactgggcagagataaaagttcttttcc

SEQ ID NO: 216 - DNA, 24 bp, synthetic construct
  misc_feature 1..24: note = synthesized sequence
  source 1..24: mol_type = other DNA
cactccaccggcggcatggacgag

SEQ ID NO: 217 - DNA, 28 bp, synthetic construct
  misc_feature 1..28: note = synthesized sequence
  source 1..28: mol_type = other DNA
cacgctgaacttgtggccgtttacgtcg

SEQ ID NO: 218 - DNA, 40 bp, synthetic construct
  misc_feature 1..40: note = synthesized sequence
  source 1..40: mol_type = other DNA
tataactagtatgaatccgcggcaggggtattccctcagc

SEQ ID NO: 219 - DNA, 73 bp, synthetic construct
  misc_feature 1..73: note = synthesized sequence
  source 1..73: mol_type = other DNA
tataggcgcgccctacttatcgtcgtcatccttgtaatctactgggcagagataaaagttcttttcctcctgg

SEQ ID NO: 220 - DNA, 42 bp, synthetic construct
  misc_feature 1..42: note = synthesized sequence
  source 1..42: mol_type = other DNA
tataactagtatggatatagaagatgaagaaaacatgagttc

SEQ ID NO: 221 - DNA, 67 bp, synthetic construct
  misc_feature 1..67: note = synthesized sequence
  source 1..67: mol_type = other DNA
tataggcgcgccctacttatcgtcgtcatccttgtaatcgggcgtgagtgagaactggtcctgctcg

SEQ ID NO: 222 - DNA, 37 bp, synthetic construct
  misc_feature 1..37: note = synthesized sequence
  source 1..37: mol_type = other DNA
tataactagtatggccgagatcaaggagaaaatctgc

SEQ ID NO: 223 - DNA, 73 bp, synthetic construct; identical to SEQ ID NO: 219
  misc_feature 1..73: note = synthesized sequence
  source 1..73: mol_type = other DNA

SEQ ID NO: 224 - DNA, 19 bp, synthetic construct
  misc_feature 1..19: note = synthesized sequence
  source 1..19: mol_type = other DNA
cgccatttcggactgggag

SEQ ID NO: 225 - DNA, 25 bp, synthetic construct
  misc_feature 1..25: note = synthesized sequence
  source 1..25: mol_type = other DNA
agagacaggtttctccatcaattac

SEQ ID NO: 226 - DNA, 16 bp, synthetic construct
  misc_feature 1..16: note = synthesized sequence
  source 1..16: mol_type = other DNA
gagcccgcgagcaacc

SEQ ID NO: 227 - DNA, 20 bp, synthetic construct
  misc_feature 1..20: note = synthesized sequence
  source 1..20: mol_type = other DNA
gcagcaggaagaagacggac

SEQ ID NO: 228 - DNA, 23 bp, synthetic construct
  misc_feature 1..23: note = synthesized sequence
  source 1..23: mol_type = other DNA
agaagcagttgaagaccagactc

SEQ ID NO: 229 - DNA, 20 bp, synthetic construct
  misc_feature 1..20: note = synthesized sequence
  source 1..20: mol_type = other DNA
ggccttcacctggaccatag

SEQ ID NO: 230 - DNA, 22 bp, synthetic construct
  misc_feature 1..22: note = synthesized sequence
  source 1..22: mol_type = other DNA
agagaagcagttgaagaccaga

SEQ ID NO: 231 - DNA, 20 bp, synthetic construct
  misc_feature 1..20: note = synthesized sequence
  source 1..20: mol_type = other DNA
cggccttcacctggaccata

SEQ ID NO: 232 - DNA, 23 bp, synthetic construct
  misc_feature 1..23: note = synthesized sequence
  source 1..23: mol_type = other DNA
cagagaagcagttgaagaccaga

SEQ ID NO: 233 - DNA, 20 bp, synthetic construct
  misc_feature 1..20: note = synthesized sequence
  source 1..20: mol_type = other DNA
cggccttcacctggaccata

SEQ ID NO: 234 - DNA, 20 bp, synthetic construct
  misc_feature 1..20: note = synthesized sequence
  source 1..20: mol_type = other DNA
tttgtgaaaggctggggacc

SEQ ID NO: 235 - DNA, 25 bp, synthetic construct
  misc_feature 1..25: note = synthesized sequence
  source 1..25: mol_type = other DNA
acaggattgtattttgtagtccacc

SEQ ID NO: 236 - DNA, 23 bp, synthetic construct
  misc_feature 1..23: note = synthesized sequence
  source 1..23: mol_type = other DNA
aggatgagttttgtgaaaggctg

SEQ ID NO: 237 - DNA, 24 bp, synthetic construct
  misc_feature 1..24: note = synthesized sequence
  source 1..24: mol_type = other DNA
attttgtagtccaccatcctgata

SEQ ID NO: 238 - DNA, 22 bp, synthetic construct
  misc_feature 1..22: note = synthesized sequence
  source 1..22: mol_type = other DNA
gatgagttttgtgaaaggctgg

SEQ ID NO: 239 - DNA, 25 bp, synthetic construct
  misc_feature 1..25: note = synthesized sequence
  source 1..25: mol_type = other DNA
attttgtagtccaccatcctgataa

SEQ ID NO: 240 - DNA, 20 bp, synthetic construct
  misc_feature 1..20: note = synthesized sequence
  source 1..20: mol_type = other DNA
cgaagagaacgagaccgcat

SEQ ID NO: 241 - DNA, 19 bp, synthetic construct
  misc_feature 1..19: note = synthesized sequence
  source 1..19: mol_type = other DNA
gaagatggtgcacaccggg

SEQ ID NO: 242 - DNA, 22 bp, synthetic construct
  misc_feature 1..22: note = synthesized sequence
  source 1..22: mol_type = other DNA
gacagatgcttcatcagcagtg

SEQ ID NO: 243 - DNA, 21 bp, synthetic construct
  misc_feature 1..21: note = synthesized sequence
  source 1..21: mol_type = other DNA
cgaacaaagccaaaccccttt

SEQ ID NO: 244 - DNA, 25 bp, synthetic construct
  misc_feature 1..25: note = synthesized sequence
  source 1..25: mol_type = other DNA
tctgttaatggacaaatagaaagcc

SEQ ID NO: 245 - DNA, 23 bp, synthetic construct
  misc_feature 1..23: note = synthesized sequence
  source 1..23: mol_type = other DNA
ggaacattcaaaggattggcact

SEQ ID NO: 246 - DNA, 20 bp, synthetic construct
  misc_feature 1..20: note = synthesized sequence
  source 1..20: mol_type = other DNA
agtcactgcagatggacgca

SEQ ID NO: 247 - DNA, 22 bp, synthetic construct
  misc_feature 1..22: note = synthesized sequence
  source 1..22: mol_type = other DNA
atctcgatgggaaattgcaggt

SEQ ID NO: 248 - DNA, 25 bp, synthetic construct
  misc_feature 1..25: note = synthesized sequence
  source 1..25: mol_type = other DNA
tcagagttttacctcatccttcttt

SEQ ID NO: 249 - DNA, 25 bp, synthetic construct
  misc_feature 1..25: note = synthesized sequence
  source 1..25: mol_type = other DNA
cctgaatacatatgatgaccttcag

SEQ ID NO: 250 - DNA, 20 bp, synthetic construct
  misc_feature 1..20: note = synthesized sequence
  source 1..20: mol_type = other DNA
agggcacagacacagacctc

SEQ ID NO: 251 - DNA, 21 bp, synthetic construct
  misc_feature 1..21: note = synthesized sequence
  source 1..21: mol_type = other DNA
agggctttcaatgccaagacg

SEQ ID NO: 252 - DNA, 19 bp, synthetic construct
  misc_feature 1..19: note = synthesized sequence
  source 1..19: mol_type = other DNA
tgacaagccaagtcctccc

SEQ ID NO: 253 - DNA, 21 bp, synthetic construct
  misc_feature 1..21: note = synthesized sequence
  source 1..21: mol_type = other DNA
attgccaatgatgagctctgg

SEQ ID NO: 254 - DNA, 25 bp, synthetic construct
  misc_feature 1..25: note = synthesized sequence
  source 1..25: mol_type = other DNA
ttatagacataagttctccttgcct

SEQ ID NO: 255 - DNA, 20 bp, synthetic construct
  misc_feature 1..20: note = synthesized sequence
  source 1..20: mol_type = other DNA
tcaatcccatggagccaaca

SEQ ID NO: 256 - DNA, 50 bp, synthetic construct
  misc_feature 1..50: note = synthesized sequence
  source 1..50: mol_type = other DNA
tacacgacgctcttccgatcttaagtagaggccgccactccaccggcggc

SEQ ID NO: 257 - DNA, 51 bp, synthetic construct
  misc_feature 1..51: note = synthesized sequence
  source 1..51: mol_type = other DNA
tacacgacgctcttccgatctatcatgcttagccgccactccaccggcggc

SEQ ID NO: 258 - DNA, 52 bp, synthetic construct
  misc_feature 1..52: note = synthesized sequence
  source 1..52: mol_type = other DNA
tacacgacgctcttccgatctgatgcacatctgccgccactccaccggcggc

SEQ ID NO: 259 - DNA, 53 bp, synthetic construct
  misc_feature 1..53: note = synthesized sequence
  source 1..53: mol_type = other DNA
tacacgacgctcttccgatctcgattgctcgacgccgccactccaccggcggc

SEQ ID NO: 260 - DNA, 54 bp, synthetic construct
  misc_feature 1..54: note = synthesized sequence
  source 1..54: mol_type = other DNA
tacacgacgctcttccgatcttcgatagcaattcgccgccactccaccggcggc

SEQ ID NO: 261 - DNA, 55 bp, synthetic construct
  misc_feature 1..55: note = synthesized sequence
  source 1..55: mol_type = other DNA
tacacgacgctcttccgatctatcgatagttgcttgccgccactccaccggcggc

SEQ ID NO: 262 - DNA, 56 bp, synthetic construct
  misc_feature 1..56: note = synthesized sequence
  source 1..56: mol_type = other DNA
tacacgacgctcttccgatctgatcgatccagttaggccgccactccaccggcggc

SEQ ID NO: 263 - DNA, 57 bp, synthetic construct
  misc_feature 1..57: note = synthesized sequence
  source 1..57: mol_type = other DNA
tacacgacgctcttccgatctcgatcgatttgagcctgccgccactccaccggcggc

SEQ ID NO: 264 - DNA, 58 bp, synthetic construct
  misc_feature 1..58: note = synthesized sequence
  source 1..58: mol_type = other DNA
tacacgacgctcttccgatctacgatcgatacacgatcgccgccactccaccggcggc

SEQ ID NO: 265 - DNA, 59 bp, synthetic construct
  misc_feature 1..59: note = synthesized sequence
  source 1..59: mol_type = other DNA
tacacgacgctcttccgatcttacgatcgatggtccagagccgccactccaccggcggc

SEQ ID NO: 266 - DNA, 50 bp, synthetic construct
  misc_feature 1..50: note = synthesized sequence
  source 1..50: mol_type = other DNA
agacgtgtgctcttccgatcttaagtagagtcgccgtccagctcgaccag

SEQ ID NO: 267 - DNA, 51 bp, synthetic construct
  misc_feature 1..51: note = synthesized sequence
  source 1..51: mol_type = other DNA
agacgtgtgctcttccgatctatcatgcttatcgccgtccagctcgaccag

SEQ ID NO: 268 - DNA, 52 bp, synthetic construct
  misc_feature 1..52: note = synthesized sequence
  source 1..52: mol_type = other DNA
agacgtgtgctcttccgatctgatgcacatcttcgccgtccagctcgaccag

SEQ ID NO: 269 - DNA, 53 bp, synthetic construct
  misc_feature 1..53: note = synthesized sequence
  source 1..53: mol_type = other DNA
agacgtgtgctcttccgatctcgattgctcgactcgccgtccagctcgaccag

SEQ ID NO: 270 - DNA, 54 bp, synthetic construct
  misc_feature 1..54: note = synthesized sequence
  source 1..54: mol_type = other DNA
agacgtgtgctcttccgatcttcgatagcaattctcgccgtccagctcgaccag

SEQ ID NO: 271 - DNA, 55 bp, synthetic construct
  misc_feature 1..55: note = synthesized sequence
  source 1..55: mol_type = other DNA
agacgtgtgctcttccgatctatcgatagttgctttcgccgtccagctcgaccag

SEQ ID NO: 272 - DNA, 56 bp, synthetic construct
  misc_feature 1..56: note = synthesized sequence
  source 1..56: mol_type = other DNA
agacgtgtgctcttccgatctgatcgatccagttagtcgccgtccagctcgaccag

SEQ ID NO: 273 - DNA, 57 bp, synthetic construct
  misc_feature 1..57: note = synthesized sequence
  source 1..57: mol_type = other DNA
agacgtgtgctcttccgatctcgatcgatttgagccttcgccgtccagctcgaccag

SEQ ID NO: 274 - DNA, 58 bp, synthetic construct
  misc_feature 1..58: note = synthesized sequence
  source 1..58: mol_type = other DNA
agacgtgtgctcttccgatctacgatcgatacacgatctcgccgtccagctcgaccag

SEQ ID NO: 275 - DNA, 59 bp, synthetic construct
  misc_feature 1..59: note = synthesized sequence
  source 1..59: mol_type = other DNA
agacgtgtgctcttccgatcttacgatcgatggtccagatcgccgtccagctcgaccag

SEQ ID NO: 276 - DNA, 18 bp, synthetic construct
  misc_feature 1..18: note = synthesized sequence
  source 1..18: mol_type = other DNA
ggggaactcgggcaacct

SEQ ID NO: 277 - DNA, 19 bp, synthetic construct
  misc_feature 1..19: note = synthesized sequence
  source 1..19: mol_type = other DNA
gaatcggatctgccccgtg

SEQ ID NO: 278 - DNA, 19 bp, synthetic construct
  misc_feature 1..19: note = synthesized sequence
  source 1..19: mol_type = other DNA
catcgaggccaagctggaa

SEQ ID NO: 279 - DNA, 20 bp, synthetic construct
  misc_feature 1..20: note = synthesized sequence
  source 1..20: mol_type = other DNA
gtagtgaggagggagacccc

SEQ ID NO: 280 - DNA, 20 bp, synthetic construct
  misc_feature 1..20: note = synthesized sequence
  source 1..20: mol_type = other DNA
aagcctccttccttccccaa

SEQ ID NO: 281 - DNA, 21 bp, synthetic construct
  misc_feature 1..21: note = synthesized sequence
  source 1..21: mol_type = other DNA
atcgatacactccctagccca

SEQ ID NO: 282 - DNA, 22 bp, synthetic construct
  misc_feature 1..22: note = synthesized sequence
  source 1..22: mol_type = other DNA
acaaattcggtacatcctcgac

SEQ ID NO: 283 - DNA, 21 bp, synthetic construct
  misc_feature 1..21: note = synthesized sequence
  source 1..21: mol_type = other DNA
ttcagccatctttggaaggtt

SEQ ID NO: 284 - DNA, 20 bp, synthetic construct
  misc_feature 1..20: note = synthesized sequence
  source 1..20: mol_type = other DNA
acgccgcattgaccatctat

SEQ ID NO: 285 - DNA, 20 bp, synthetic construct
  misc_feature 1..20: note = synthesized sequence
  source 1..20: mol_type = other DNA
tagccaggaggttctcaaca

SEQ ID NO: 286 - DNA, 21 bp, synthetic construct
  misc_feature 1..21: note = synthesized sequence
  source 1..21: mol_type = other DNA
ggcatggactgtggtcatgag

SEQ ID NO: 287 - DNA, 20 bp, synthetic construct
  misc_feature 1..20: note = synthesized sequence
  source 1..20: mol_type = other DNA
tgcaccaccaactgcttagc

SEQ ID NO: 288 - DNA, 22 bp, synthetic construct
  misc_feature 1..22: note = synthesized sequence
  source 1..22: mol_type = other DNA
ccccgtaatgcagaagaagacc

SEQ ID NO: 289 - DNA, 21 bp, synthetic construct
  misc_feature 1..21: note = synthesized sequence
  source 1..21: mol_type = other DNA
gtccttcagcttcagcctctg

SEQ ID NO: 290 - DNA, 20 bp, synthetic construct
  misc_feature 1..20: note = synthesized sequence
  source 1..20: mol_type = other DNA
aacgcaacatgaaggtgctc

SEQ ID NO: 291 - DNA, 20 bp, synthetic construct
  misc_feature 1..20: note = synthesized sequence
  source 1..20: mol_type = other DNA
accttgacggtgactttggg

SEQ ID NO: 292 - DNA, 20 bp, synthetic construct
  misc_feature 1..20: note = synthesized sequence
  source 1..20: mol_type = other DNA
cagtgcaatgagggaccagt

SEQ ID NO: 293 - DNA, 24 bp, synthetic construct
  misc_feature 1..24: note = synthesized sequence
  source 1..24: mol_type = other DNA
aggaccataggtacatcttcagag

SEQ ID NO: 294 - DNA, 22 bp, synthetic construct
  misc_feature 1..22: note = synthesized sequence
  source 1..22: mol_type = other DNA
cgaacgagttgtatcacctgga

SEQ ID NO: 295 - DNA, 20 bp, synthetic construct
  misc_feature 1..20: note = synthesized sequence
  source 1..20: mol_type = other DNA
cgatggctgtccctcaaagt

SEQ ID NO: 296 - DNA, 23 bp, synthetic construct
  misc_feature 1..23: note = synthesized sequence
  source 1..23: mol_type = other DNA
agttgctcttttcactcaaggtc

SEQ ID NO: 297 - DNA, 21 bp, synthetic construct
  misc_feature 1..21: note = synthesized sequence
  source 1..21: mol_type = other DNA
ttctctctgagttcagacgct

SEQ ID NO: 298 - DNA, 52 bp, synthetic construct
  misc_feature 1..52: note = synthesized sequence
  source 1..52: mol_type = other DNA
tacacgacgctcttccgatcttaagtagagtggcacaggaggaaagagcatc

SEQ ID NO: 299 - DNA, 49 bp, synthetic construct
  misc_feature 1..49: note = synthesized sequence
  source 1..49: mol_type = other DNA
agacgtgtgctcttccgatcttaagtagaggcaccacctccatgccctc

SEQ ID NO: 300 - DNA, 49 bp, synthetic construct
  misc_feature 1..49: note = synthesized sequence
  source 1..49: mol_type = other DNA
tacacgacgctcttccgatcttaagtagagcatcgcagactgcggcaag

SEQ ID NO: 301 - DNA, 52 bp, synthetic construct
  misc_feature 1..52: note = synthesized sequence
  source 1..52: mol_type = other DNA
agacgtgtgctcttccgatcttaagtagagagtccatgggcctgtggaatgt

SEQ ID NO: 302 - DNA, 19 bp, synthetic construct
  misc_feature 1..19: note = synthesized sequence
  source 1..19: mol_type = other DNA
gaaaaactggcccgagagc

SEQ ID NO: 303 - DNA, 20 bp, synthetic construct
  misc_feature 1..20: note = synthesized sequence
  source 1..20: mol_type = other DNA
ctgagtctgggctgagggac

SEQ ID NO: 304 - DNA, 20 bp, synthetic construct
  misc_feature 1..20: note = synthesized sequence
  source 1..20: mol_type = other DNA
cgcttccaggtcaacaacac

SEQ ID NO: 305 - DNA, 19 bp, synthetic construct
  misc_feature 1..19: note = synthesized sequence
  source 1..19: mol_type = other DNA
ctcgcgtagatcagcaccg

SEQ ID NO: 306 - DNA, 21 bp, synthetic construct
  misc_feature 1..21: note = synthesized sequence
  source 1..21: mol_type = other DNA
cccctctgagtcaggaaacat

SEQ ID NO: 307 - DNA, 19 bp, synthetic construct
  misc_feature 1..19: note = synthesized sequence
  source 1..19: mol_type = other DNA
gaagatgacaggggccagg

SEQ ID NO: 308 - DNA, 19 bp, synthetic construct
  misc_feature 1..19: note = synthesized sequence
  source 1..19: mol_type = other DNA
tagcactggctggaatgag

SEQ ID NO: 309 - DNA, 21 bp, synthetic construct
  misc_feature 1..21: note = synthesized sequence
  source 1..21: mol_type = other DNA
gtttcggaggtaacctgtaag

SEQ ID NO: 310 - DNA, 20 bp, synthetic construct
  misc_feature 1..20: note = synthesized sequence
  source 1..20: mol_type = other DNA
tacagcaaccatgagtacaa

SEQ ID NO: 311 - DNA, 19 bp, synthetic construct
  misc_feature 1..19: note = synthesized sequence
  source 1..19: mol_type = other DNA
tcaggtgtttcacataggc

SEQ ID NO: 312 - DNA, 19 bp, synthetic construct
  misc_feature 1..19: note = synthesized sequence
  source 1..19: mol_type = other DNA
ctgcaaccatgagtgagaa

SEQ ID NO: 313 - DNA, 21 bp, synthetic construct
  misc_feature 1..21: note = synthesized sequence
  source 1..21: mol_type = other DNA
cctttgaggtgctttagatag

SEQ ID NO: 314 - DNA, 19 bp, synthetic construct
  misc_feature 1..19: note = synthesized sequence
  source 1..19: mol_type = other DNA
gccctgagaaaggagacat

SEQ ID NO: 315 - DNA, 24 bp, synthetic construct
  misc_feature 1..24: note = synthesized sequence
  source 1..24: mol_type = other DNA
ctgttctggaggtactctaggtat

SEQ ID NO: 316 - DNA, 18 bp, synthetic construct
  misc_feature 1..18: note = synthesized sequence
  source 1..18: mol_type = other DNA
tttgaagagggctgagaa

SEQ ID NO: 317 - DNA, 19 bp, synthetic construct
  misc_feature 1..19: note = synthesized sequence
  source 1..19: mol_type = other DNA
tgttctggatatttcatgg

SEQ ID NO: 318 - DNA, 20 bp, synthetic construct
  misc_feature 1..20: note = synthesized sequence
  source 1..20: mol_type = other DNA
catctgcctccccatattcc

SEQ ID NO: 319 - DNA, 22 bp, synthetic construct
  misc_feature 1..22: note = synthesized sequence
  source 1..22: mol_type = other DNA
tccatcctagctcatctccaaa

SEQ ID NO: 320 - DNA, 18 bp, synthetic construct
  misc_feature 1..18: note = synthesized sequence
  source 1..18: mol_type = other DNA
tgctccagaaggccagac

SEQ ID NO: 321 - DNA, 25 bp, synthetic construct
  misc_feature 1..25: note = synthesized sequence
  source 1..25: mol_type = other DNA
ttcataaatactactaaggcacagg

SEQ ID NO: 322 - DNA, 21 bp, synthetic construct
  misc_feature 1..21: note = synthesized sequence
  source 1..21: mol_type = other DNA
acagatgaagtgctccttcca

SEQ ID NO: 323 - DNA, 21 bp, synthetic construct
  misc_feature 1..21: note = synthesized sequence
  source 1..21: mol_type = other DNA
gtcggagattcgtagctggat

SEQ ID NO: 324 - DNA, 21 bp, synthetic construct
  misc_feature 1..21: note = synthesized sequence
  source 1..21: mol_type = other DNA
cattgtggccaaggagatctg

SEQ ID NO: 325 - DNA, 21 bp, synthetic construct
  misc_feature 1..21: note = synthesized sequence
  source 1..21: mol_type = other DNA
cttcggagtttgggtttgctt

SEQ ID NO: 326 - DNA, 20 bp, synthetic construct
  misc_feature 1..20: note = synthesized sequence
  source 1..20: mol_type = other DNA
catcacttgctgctgacacg

SEQ ID NO: 327 - DNA, 18 bp, synthetic construct
  misc_feature 1..18: note = synthesized sequence
  source 1..18: mol_type = other DNA
tgtggaatctgccgggag

SEQ ID NO: 328 - DNA, 18 bp, synthetic construct
  misc_feature 1..18: note = synthesized sequence
  source 1..18: mol_type = other DNA
ctgactctaagtggcatt

SEQ ID NO: 329 - DNA, 18 bp, synthetic construct
  misc_feature 1..18: note = synthesized sequence
  source 1..18: mol_type = other DNA
tgatggccttcgattctg

SEQ ID NO: 330 - DNA, 23 bp, synthetic construct
  misc_feature 1..23: note = synthesized sequence
  source 1..23: mol_type = other DNA
cggagtcaacggatttggtcgta

SEQ ID NO: 331 - DNA, 24 bp, synthetic construct
  misc_feature 1..24: note = synthesized sequence
  source 1..24: mol_type = other DNA
agccttctccatggtggtgaagac

SEQ ID NO: 332 - DNA, 2820 bp, synthetic construct
  misc_feature 1..2820: note = synthesized sequence
  source 1..2820: mol_type = other DNA
atggccgagatcaaggagaaaatctgcgactatctcttcaatgtgtctgactcctctgccctgaatttggctaaaaatattggccttaccaaggcccgagatataaatgctgtgctaattgacatggaaaggcagggggatgtctatagacaagggacaacccctcccatatggcatttgacagacaagaagcgagagaggatgcaaatcaagagaaatacgaacagtgttcctgaaaccgctccagctgcaatccctgagaccaaaagaaacgcagagttcctcacctgtaatatacccacatcaaatgcctcaaataacatggtaaccacagaaaaagtggagaatgggcaggaacctgtcataaagttagaaaacaggcaagaggccagaccagaaccagcaagactgaaaccacctgttcattacaatggcccctcaaaagcagggtatgttgactttgaaaatggccagtgggccacagatgacatcccagatgacttgaatagtatccgcgcagcaccaggtgagtttcgagccatcatggagatgccctccttctacagtcatggcttgccacggtgttcaccctacaagaaactgacagagtgccagctgaagaaccccatcagcgggctgttagaatatgcccagttcgctagtcaaacctgtgagttcaacatgatagagcagagtggaccaccccatgaacctcgatttaaattccaggttgtcatcaatggccgagagtttcccccagctgaagctggaagcaagaaagtggccaagcaggatgcagctatgaaagccatgacaattctgctagaggaagccaaagccaaggacagtggaaaatcagaagaatcatcccactattccacagagaaagaatcagagaagactgcagagtcccagacccccaccccttcagccacatccttcttttctgggaagagccccgtcaccacactgcttgagtgtatgcacaaattggggaactcctgcgaattccgtctcctgtccaaagaaggccctgcccatgaacccaagttccaatactgtgttgcagtgggagcccaaactttccccagtgtgagtgctcccagcaagaaagtggcaaagcagatggccgcagaggaagccatgaaggccctgcatggggaggcgaccaactccatggcttctgataaccagcctgaaggtatgatctcagagtcacttgataacttggaatccatgatgcccaacaaggtcaggaagattggcgagctcgtgagatacctgaacaccaaccctgtgggtggccttttggagtacgcccgctcccatggctttgctgctgaattcaagttggtcgaccagtccggacctcctcacgagcccaagttcgtttaccaagcaaaagttgggggtcgctggttcccagccgtctgcgcacacagcaagaagcaaggcaagcaggaagcagcagatgcggctctccgtgtcttgattggggagaacgagaaggcagaacgcatgggtttcacagaggtaaccccagtgacaggggccagtctcagaagaactatgctcctcctctcaaggtccccagaagcacagccaaagacactccctctcactggcagcaccttccatgaccagatagccatgctgagccaccggtgcttcaacactctgactaacagcttccagccctccttgctcggccgcaagattctggccgccatcattatgaaaaaagactctgaggacatgggtgtcgtcgtcagcttgggaacagggaatcgctgtgtaaaaggagattctctcagcctaaaaggagaaactgtcaatgactgccatgcagaaataatctcccggagaggcttcatcaggtttctctacagtgagttaatgaaatacaactcccagactgcgaaggatagtatatttgaacctgctaagggaggagaaaagctccaaataaaaaagactgtgtcattccatctgtatatcagcactgctccgtgtggagatggcgccctctttgacaagtcctgcagcgaccgtgctatggaaagcacagaatcccgccactaccctgtcttcgagaatcccaaacaaggaaagctccgcaccaaggtggagaacggagaaggcacaatccctgtggaatccagtgacattgtgcctacgtgggatggcattcggctcggggagagactccgtaccatgtcctgtagtgacaaaatcctacgctggaacgtgctgggcctgcaaggggcactgttgacccacttcctgcagcccatttatctcaaatctgtcacattgggttaccttttcagccaagggcatctgacccgtgctatttgctgtcgtgtgacaagagatgggagtgcatttgaggatggactacgacatccctttattgtcaaccaccccaaggttggcagagtcagcatatatgattccaaaaggcaatccgggaagactaaggagacaagcgtcaactggtgtctggctgatggctatgacctggagatcctggacggtaccagaggcactgtggatgggccacggaatgaattgtcccgggtctccaaaaagaacatttttcttctatttaagaagctctgctccttccgttaccgcagggatctactgagactctcctatggtgaggccaagaaagctgcccgtgactacgagacggccaagaactacttcaaaaaaggcctgaaggatatgggctatgggaactggattagcaaaccccaggaggaaaagaacttttatctctgcccagtagattacaaggatgacgacgataagtag

SEQ ID NO: 333 - DNA, 3705 bp, synthetic construct
  misc_feature 1..3705: note = synthesized sequence
  source 1..3705: mol_type = other DNA
atgaatccgcggcaggggtattccctcagcggatactacacccatccatttcaaggctatgagcacagacagctcagataccagcagcctgggccaggatcttcccccagtagtttcctgcttaagcaaatagaatttctcaaggggcagctcccagaagcaccggtgattggaaagcagacaccgtcactgccaccttccctcccaggactccggccaaggtttccagtactacttgcctccagtaccagaggcaggcaagtggacatcaggggtgtccccaggggcgtgcatctcggaagtcaggggctccagagagggttccagcatccttcaccacgtggcaggagtctgccacagagaggtgttgattgcctttcctcacatttccaggaactgagtatctaccaagatcaggaacaaaggatcttaaagttcctggaagagcttggggaagggaaggccaccacagcacatgatctgtctgggaaacttgggactccgaagaaagaaatcaatcgagttttatactccctggcaaagaagggcaagctacagaaagaggcaggaacaccccctttgtggaaaatcgcggtctccactcaggcttggaaccagcacagcggagtggtaagaccagacggtcatagccaaggagccccaaactcagacccgagtttggaaccggaagacagaaactccacatctgtctcagaagatcttcttgagccttttattgcagtctcagctcaggcttggaaccagcacagcggagtggtaagaccagacagtcatagccaaggatccccaaactcagacccaggtttggaacctgaagacagcaactccacatctgccttggaagatcctcttgagtttttagacatggccgagatcaaggagaaaatctgcgactatctcttcaatgtgtctgactcctctgccctgaatttggctaaaaatattggccttaccaaggcccgagatataaatgctgtgctaattgacatggaaaggcagggggatgtctatagacaagggacaacccctcccatatggcatttgacagacaagaagcgagagaggatgcaaatcaagagaaatacgaacagtgttcctgaaaccgctccagctgcaatccctgagaccaaaagaaacgcagagttcctcacctgtaatatacccacatcaaatgcctcaaataacatggtaaccacagaaaaagtggagaatgggcaggaacctgtcataaagttagaaaacaggcaagaggccagaccagaaccagcaagactgaaaccacctgttcattacaatggcccctcaaaagcagggtatgttgactttgaaaatggccagtgggccacagatgacatcccagatgacttgaatagtatccgcgcagcaccaggtgagtttcgagccatcatggagatgccctccttctacagtcatggcttgccacggtgttcaccctacaagaaactgacagagtgccagctgaagaaccccatcagcgggctgttagaatatgcccagttcgctagtcaaacctgtgagttcaacatgatagagcagagtggaccaccccatgaacctcgatttaaattccaggttgtcatcaatggccgagagtttcccccagctgaagctggaagcaagaaagtggccaagcaggatgcagctatgaaagccatgacaattctgctagaggaagccaaagccaaggacagtggaaaatcagaagaatcatcccactattccacagagaaagaatcagagaagactgcagagtcccagacccccaccccttcagccacatccttcttttctgggaagagccccgtcaccacactgcttgagtgtatgcacaaattggggaactcctgcgaattccgtctcctgtccaaagaaggccctgcccatgaacccaagttccaatactgtgttgcagtgggagcccaaactttccccagtgtgagtgctcccagcaagaaagtggcaaagcagatggccgcagaggaagccatgaaggccctgcatggggaggcgaccaactccatggcttctgataaccagcctgaaggtatgatctcagagtcacttgataacttggaatccatgatgcccaacaaggtcaggaagattggcgagctcgtgagatacctgaacaccaaccctgtgggtggccttttggagtacgcccgctcccatggctttgctgctgaattcaagttggtcgaccagtccggacctcctcacgagcccaagttcgtttaccaagcaaaagttgggggtcgctggttcccagccgtctgcgcacacagcaagaagcaaggcaagcaggaagcagcagatgcggctctccgtgtcttgattggggagaacgagaaggcagaacgcatgggtttcacagaggtaaccccagtgacaggggccagtctcagaagaactatgctcctcctctcaaggtccccagaagcacagccaaagacactccctctcactggcagcaccttccatgaccagatagccatgctgagccaccggtgcttcaacactctgactaacagcttccagccctccttgctcggccgcaagattctggccgccatcattatgaaaaaagactctgaggacatgggtgtcgtcgtcagcttgggaacagggaatcgctgtgtaaaaggagattctctcagcctaaaaggagaaactgtcaatgactgccatgcagaaataatctcccggagaggcttcatcaggtttctctacagtgagttaatgaaatacaactcccagactgcgaaggatagtatatttgaacctgctaagggaggagaaaagctccaaataaaaaagactgtgtcattccatctgtatatcagcactgctccgtgtggagatggcgccctctttgacaagtcctgcagcgaccgtgctatggaaagcacagaatcccgccactaccctgtcttcgagaatcccaaacaaggaaagctccgcaccaaggtggagaacggagaaggcacaatccctgtggaatccagtgacattgtgcctacgtgggatggcattcggctcggggagagactccgtaccatgtcctgtagtgacaaaatcctacgctggaacgtgctgggcctgcaaggggcactgttgacccacttcctgcagcccatttatctcaaatctgtcacattgggttaccttttcagccaagggcatctgacccgtgctatttgctgtcgtgtgacaagagatgggagtgcatttgaggatggactacgacatccctttattgtcaaccaccccaaggttggcagagtcagcatatatgattccaaaaggcaatccgggaagactaaggagacaagcgtcaactggtgtctggctgatggctatgacctggagatcctggacggtaccagaggcactgtggatgggccacggaatgaattgtcccgggtctccaaaaagaacatttttcttctatttaagaagctctgctccttccgttaccgcagggatctactgagactctcctatggtgaggccaagaaagctgcccgtgactacgagacggccaagaactacttcaaaaaaggcctgaaggatatgggctatgggaactggattagcaaaccccaggaggaaaagaacttttatctctgcccagtagattacaaggatgacgacgataagtag

SEQ ID NO: 334 - DNA, 2130 bp, synthetic construct
  misc_feature 1..2130: note = synthesized sequence
  source 1..2130: mol_type = other DNA
atggatatagaagatgaagaaaacatgagttccagcagcactgatgtgaaggaaaaccgcaatctggacaacgtgtcccccaaggatggcagcacacctgggcctggcgagggctctcagctctccaatgggggtggtggtggccccggcagaaagcggcccctggaggagggcagcaatggccactccaagtaccgcctgaagaaaaggaggaaaacaccagggcccgtcctccccaagaacgccctgatgcagctgaatgagatcaagcctggtttgcagtacacactcctgtcccagactgggcccgtgcacgcgcctttgtttgtcatgtctgtggaggtgaatggccaggtttttgagggctctggtcccacaaagaaaaaggcaaaactccatgctgctgagaaggccttgaggtctttcgttcagtttcctaatgcctctgaggcccacctggccatggggaggaccctgtctgtcaacacggacttcacatctgaccaggccgacttccctgacacgctcttcaatggttttgaaactcctgacaaggcggagcctcccttttacgtgggctccaatggggatgactccttcagttccagcggggacctcagcttgtctgcttccccggtgcctgccagcctagcccagcctcctctccctgccttaccaccattcccacccccgagtgggaagaatcccgtgatgatcttgaacgaactgcgcccaggactcaagtatgacttcctctccgagagcggggagagccatgccaagagcttcgtcatgtctgtggtcgtggatggtcagttctttgaaggctcggggagaaacaagaagcttgccaaggcccgggctgcgcagtctgccctggccgccatttttaacttgcacttggatcagacgccatctcgccagcctattcccagtgagggtcttcagctgcatttaccgcaggttttagctgacgctgtctcacgcctggtcctgggtaagtttggtgacctgaccgacaacttctcctcccctcacgctcgcagaaaagtgctggctggagtcgtcatgacaacaggcacagatgttaaagatgccaaggtgataagtgtttctacaggaacaaaatgtattaatggtgaatacatgagtgatcgtggccttgcattaaatgactgccatgcagaaataatatctcggagatccttgctcagatttctttatacacaacttgagctttacttaaataacaaagatgatcaaaaaagatccatctttcagaaatcagagcgaggggggtttaggctgaaggagaatgtccagtttcatctgtacatcagcacctctccctgtggagatgccagaatcttctcaccacatgagccaatcctggaagaaccagcagatagacacccaaatcgtaaagcaagaggacagctacggaccaaaatagagtctggtgaggggacgattccagtgcgctccaatgcgagcatccaaacgtgggacggggtgctgcaaggggagcggctgctcaccatgtcctgcagtgacaagattgcacgctggaacgtggtgggcatccagggatccctgctcagcattttcgtggagcccatttacttctcgagcatcatcctgggcagcctttaccacggggaccacctttccagggccatgtaccagcggatctccaacatagaggacctgccacctctctacaccctcaacaagcctttgctcagtggcatcagcaatgcagaagcacggcagccagggaaggcccccaacttcagtgtcaactggacggtaggcgactccgctattgaggtcatcaacgccacgactgggaaggatgagctgggccgcgcgtcccgcctgtgtaagcacgcgttgtactgtcgctggatgcgtgtgcacggcaaggttccctcccacttactacgctccaagattaccaaacccaacgtgtaccatgagtccaagctggcggcaaaggagtaccaggccgccaaggcgcgtctgttcacagccttcatcaaggcggggctgggggcctgggtggagaagcccaccgagcaggaccagttctcactcacgcccgattacaaggatgacgacgataagtag

SEQ ID NO: 335 - DNA, 4401 bp, synthetic construct
  misc_feature 1..4401: note = synthesized sequence
  source 1..4401: mol_type = other DNA
atgatgagctttgtgcaaaaggggagctggctacttctcgctctgcttcatcccactattattttggcacaacaggaagctgttgaaggaggatgttcccatcttggtcagtcctatgcggatagagatgtctggaagccagaaccatgccaaatatgtgtctgtgactcaggatccgttctctgcgatgacataatatgtgacgatcaagaattagactgccccaacccagaaattccatttggagaatgttgtgcagtttgcccacagcctccaactgctcctactcgccctcctaatggtcaaggacctcaaggccccaagggagatccaggccctcctggtattcctgggagaaatggtgaccctggtattccaggacaaccagggtcccctggttctcctggcccccctggaatctgtgaatcatgccctactggtcctcagaactattctccccagtatgattcatatgatgtcaagtctggagtagcagtaggaggactcgcaggctatcctggaccagctggccccccaggccctcccggtccccctggtacatctggtcatcctggttcccctggatctccaggataccaaggaccccctggtgaacctgggcaagctggtccttcaggccctccaggacctcctggtgctataggtccatctggtcctgctggaaaagatggagaatcaggtagacccggacgacctggagagcgaggattgcctggacctccaggtatcaaaggtccagctgggatacctggattccctggtatgaaaggacacagaggcttcgatggacgaaatggagaaaagggtgaaacaggtgctcctggattaaagggtgaaaatggtcttccaggcgaaaatggagctcctggacccatgggtccaagaggggctcctggtgagcgaggacggccaggacttcctggggctgcaggtgctcggggtaatgacggtgctcgaggcagtgatggtcaaccaggccctcctggtcctcctggaactgccggattccctggatcccctggtgctaagggtgaagttggacctgcagggtctcctggttcaaatggtgcccctggacaaagaggagaacctggacctcagggacacgctggtgctcaaggtcctcctggccctcctgggattaatggtagtcctggtggtaaaggcgaaatgggtcccgctggcattcctggagctcctggactgatgggagcccggggtcctccaggaccagccggtgctaatggtgctcctggactgcgaggtggtgcaggtgagcctggtaagaatggtgccaaaggagagcccggaccacgtggtgaacgcggtgaggctggtattccaggtgttccaggagctaaaggcgaagatggcaaggatggatcacctggagaacctggtgcaaatgggcttccaggagctgcaggagaaaggggtgcccctgggttccgaggacctgctggaccaaatggcatcccaggagaaaagggtcctgctggagagcgtggtgctccaggccctgcagggcccagaggagctgctggagaacctggcagagatggcgtccctggaggtccaggaatgaggggcatgcccggaagtccaggaggaccaggaagtgatgggaaaccagggcctcccggaagtcaaggagaaagtggtcgaccaggtcctcctgggccatctggtccccgaggtcagcctggtgtcatgggcttccccggtcctaaaggaaatgatggtgctcctggtaagaatggagaacgaggtggccctggaggacctggccctcagggtcctcctggaaagaatggtgaaactggacctcagggacccccagggcctactgggcctggtggtgacaaaggagacacaggaccccctggtccacaaggattacaaggcttgcctggtacaggtggtcctccaggagaaaatggaaaacctggggaaccaggtccaaagggtgatgccggtgcacctggagctccaggaggcaagggtgatgctggtgcccctggtgaacgtggacctcctggattggcaggggccccaggacttagaggtggagctggtccccctggtcccgaaggaggaaagggtgctgctggtcctcctgggccacctggtgctgctggtactcctggtctgcaaggaatgcctggagaaagaggaggtcttggaagtcctggtccaaagggtgacaagggtgaaccaggcggtccaggtgctgatggtgtcccagggaaagatggcccaaggggtcctactggtcctattggtcctcctggcccagctggccagcctggagataagggtgaaggtggtgcccccggacttccaggtatagctggacctcgtggtagccctggtgagagaggtgaaactggccctccaggacctgctggtttccctggtgctcctggacagaatggtgaacctggtggtaaaggagaaagaggggctccgggtgagaaaggtgaaggaggccctcctggagttgcaggaccccctggaggttctggacctgctggtcctcctggtccccaaggtgtcaaaggtgaacgtggcagtcctggtggacctggtgctgctggcttccctggtgctcgtggtcttcctggtcctcctggtagtaatggtaacccaggacccccaggtcccagcggttctccaggcaaggatgggcccccaggtcctgcgggtaacactggtgctcctggcagccctggagtgtctggaccaaaaggtgatgctggccaaccaggagagaagggatcgcctggtgcccagggcccaccaggagctccaggcccacttgggattgctgggatcactggagcacggggtcttgcaggaccaccaggcatgccaggtcctaggggaagccctggccctcagggtgtcaagggtgaaagtgggaaaccaggagctaacggtctcagtggagaacgtggtccccctggaccccagggtcttcctggtctggctggtacagctggtgaacctggaagagatggaaaccctggatcagatggtcttccaggccgagatggatctcctggtggcaagggtgatcgtggtgaaaatggctctcctggtgcccctggcgctcctggtcatccaggcccacctggtcctgtcggtccagctggaaagagtggtgacagaggagaaagtggccctgctggccctgctggtgctcccggtcctgctggttcccgaggtgctcctggtcctcaaggcccacgtggtgacaaaggtgaaacaggtgaacgtggagctgctggcatcaaaggacatcgaggattccctggtaatccaggtgccccaggttctccaggccctgctggtcagcagggtgcaatcggcagtccaggacctgcaggccccagaggacctgttggacccagtggacctcctggcaaagatggaaccagtggacatccaggtcccattggaccaccagggcctcgaggtaacagaggtgaaagaggatctgagggctccccaggccacccagggcaaccaggccctcctggacctcctggtgcccctggtccttgctgtggtggtgttggagccgctgccattgctgggattggaggtgaaaaagctggcggttttgccccgtattatggagatgaaccaatggatttcaaaatcaacaccgatgagattatgacttcactcaagtctgttaatggacaaatagaaagcctcattagtcctgatggttctcgtaaaaaccccgctagaaactgcagagacctgaaattctgccatcctgaactcaagagtggagaatactgggttgaccctaaccaaggatgcaaattggatgctatcaaggtattctgtaatatggaaactggggaaacatgcataagtgccaatcctttgaatgttccacggaaacactggtggacagattctagtgctgagaagaaacacgtttggtttggagagtccatggatggtggttttcagtttagctacggcaatcctgaacttcctgaagatgtccttgatgtgcagctggcattccttcgacttctctccagccgagcttcccagaacatcacatatcactgcaaaaatagcattgcatacatggatcaggccagtggaaatgtaaagaaggccctgaagctgatggggtcaaatgaaggtgaattcaaggctgaaggaaatagcaaattcacctacacagttctggaggatggttgcacgaaacacactggggaatggagcaaaacagtctttgaatatcgaacacgcaaggctgtgagactacctattgtagatattgcaccctatgacattggtggtcctgatcaagaatttggtgtggacgttggccctgtttgctttttataa

SEQ ID NO: 336 - DNA, 3117 bp, synthetic construct
  misc_feature 1..3117: note = synthesized sequence
  source 1..3117: mol_type = other DNA
atgacttcctcgctgcagcggccctggcgggtgccctggctaccatggaccatcctgctggtcagcgctgcggctgcttcgcagaatcaagaacggctatgtgcgtttaaagatccgtatcagcaagaccttgggataggtgagagtagaatctctcatgaaaatgggacaatattatgctcgaaaggtagcacctgctatggcctttgggagaaatcaaaaggggacataaatcttgtaaaacaaggatgttggtctcacattggagatccccaagagtgtcactatgaagaatgtgtagtaactaccactcctccctcaattcagaatggaacataccgtttctgctgttgtagcacagatttatgtaatgtcaactttactgagaattttccacctcctgacacaacaccactcagtccacctcattcatttaaccgagatgagacaataatcattgctttggcatcagtctctgtattagctgttttgatagttgccttatgctttggatacagaatgttgacaggagaccgtaaacaaggtcttcacagtatgaacatgatggaggcagcagcatccgaaccctctcttgatctagataatctgaaactgttggagctgattggccgaggtcgatatggagcagtatataaaggctccttggatgagcgtccagttgctgtaaaagtgttttcctttgcaaaccgtcagaattttatcaacgaaaagaacatttacagagtgcctttgatggaacatgacaacattgcccgctttatagttggagatgagagagtcactgcagatggacgcatggaatatttgcttgtgatggagtactatcccaatggatctttatgcaagtatttaagtctccacacaagtgactgggtaagctcttgccgtcttgctcattctgttactagaggactggcttatcttcacacagaattaccacgaggagatcattataaacctgcaatttcccatcgagatttaaacagcagaaatgtcctagtgaaaaatgatggaacctgtgttattagtgactttggactgtccatgaggctgactggaaatagactggtgcgcccaggggaggaagataatgcagccataagcgaggttggcactatcagatatatggcaccagaagtgctagaaggagctgtgaacttgagggactgtgaatcagctttgaaacaagtagacatgtatgctcttggactaatctattgggagatatttatgagatgtacagacctcttcccaggggaatccgtaccagagtaccagatggcttttcagacagaggttggaaaccatcccacttttgaggatatgcaggttctcgtgtctagggaaaaacagagacccaagttcccagaagcctggaaagaaaatagcctggcagtgaggtcactcaaggagacaatcgaagactgttgggaccaggatgcagaggctcggcttactgcacagtgtgctgaggaaaggatggctgaacttatgatgatttgggaaagaaacaaatctgtgagcccaacagtcaatccaatgtctactgctatgcagaatgaacgcaacctgtcacataataggcgtgtgccaaaaattggtccttatccagattattcttcctcctcatacattgaagactctatccatcatactgacagcatcgtgaagaatatttcctctgagcattctatgtccagcacacctttgactataggggaaaaaaaccgaaattcaattaactatgaacgacagcaagcacaagctcgaatccccagccctgaaacaagtgtcaccagcctctccaccaacacaacaaccacaaacaccacaggactcacgccaagtactggcatgactactatatctgagatgccatacccagatgaaacaaatctgcataccacaaatgttgcacagtcaattgggccaacccctgtctgcttacagctgacagaagaagacttggaaaccaacaagctagacccaaaagaagttgataagaacctcaaggaaagctctgatgagaatctcatggagcactctcttaaacagttcagtggcccagacccactgagcagtactagttctagcttgctttacccactcataaaacttgcagtagaagcaactggacagcaggacttcacacagactgcaaatggccaagcatgtttgattcctgatgttctgcctactcagatctatcctctccccaagcagcagaaccttcccaagagacctactagtttgcctttgaacaccaaaaattcaacaaaagagccccggctaaaatttggcagcaagcacaaatcaaacttgaaacaagtcgaaactggagttgccaagatgaatacaatcaatgcagcagaacctcatgtggtgacagtcaccatgaatggtgtggcaggtagaaaccacagtgttaactcccatgctgccacaacccaatatgccaatgggacagtactatctggccaaacaaccaacatagtgacacatagggcccaagaaatgttgcagaatcagtttattggtgaggacacccggctgaatattaattccagtcctgatgagcatgagcctttactgagacgagagcaacaagctggccatgatgaaggtgttctggatcgtcttgtggacaggagggaacggccactagaaggtggccgaactaattccaataacaacaacagcaatccatgttcagaacaagatgttcttgcacagggtgttccaagcacagcagcagatcctgggccatcaaagcccagaagagcacagaggcctaattctctggatctttcagccacaaatgtcctggatggcagcagtatacagataggtgagtcaacacaagatggcaaatcaggatcaggtgaaaagatcaagaaacgtgtgaaaactccctattctcttaagcggtggcgcccctccacctgggtcatctccactgaatcgctggactgtgaagtcaacaataatggcagtaacagggcagttcattccaaatccagcactgctgtttaccttgcagaaggaggcactgctacaaccatggtgtctaaagatataggaatgaactgtctgtga

SEQ ID NO: 337 - DNA, 3590 bp, synthetic construct
  misc_feature 1..3590: note = synthesized sequence
  source 1..3590: mol_type = other DNA
atgcctacagctgagagtgaagcaaaagtaaaaaccaaagttcgctttgaagaattgcttaagacccacagtgatctaatgcgtgaaaagaaaaaactgaagaaaaaacttgtcaggtctgaagaaaacatctcacctgacactattagaagcaatcttcactatatgaaagaaactacaagtgatgatcccgacactattagaagcaatcttccccatattaaagaaactacaagtgatgatgtaagtgctgctaacactaacaacctgaagaagagcacgagagtcactaaaaacaaattgaggaacacacagttagcaactgaaaatcctaatggtgatgctagtgtagaggaagacaaacaaggaaagccaaataaaaaggtgataaagacggtgccccagttgactacacaagacctgaaaccggaaactcctgagaataaggttgattctacacaccagaaaacacatacaaagccacagccaggcgttgatcatcagaaaagtgagaaggcaaatgagggaagagaagagactgatttagaagaggatgaagaattgatgcaagcatatcagtgccatgtaactgaagaaatggcaaaggagattaagaggaaaataagaaagaaactgaaagaacagttgacttactttccctcagatactttattccatgatgacaaactaagcagtgaaaaaaggaaaaagaaaaaggaagttccagtcttctctaaagctgaaacaagtacattgaccatctctggtgacacagttgaaggtgaacaaaagaaagaatcttcagttagatcagtttcttcagattctcatcaagatgatgaaataagctcaatggaacaaagcacagaagacagcatgcaagatgatacaaaacctaaaccaaaaaaaacaaaaaagaagactaaagcagttgcagataataatgaagatgttgatggtgatggtgttcatgaaataacaagccgagatagcccggtttatcccaaatgtttgcttgatgatgaccttgtcttgggagtttacattcaccgaactgatagacttaagtcagattttatgatttctcacccaatggtaaaaattcatgtggttgatgagcatactggtcaatatgtcaagaaagatgatagtggacggcctgtttcatcttactatgaaaaagagaatgtggattatattcttcctattatgacccagccatatgattttaaacagttaaaatcaagacttccagagtgggaagaacaaattgtatttaatgaaaattttccctatttgcttcgaggctctgatgagagtcctaaagtcatcctgttctttgagattcttgatttcttaagcgtggatgaaattaagaataattctgaggttcaaaaccaagaatgtggctttcggaaaattgcctgggcatttcttaagcttctgggagccaatggaaatgcaaacatcaactcaaaacttcgcttgcagctatattacccacctactaagcctcgatccccattaagtgttgttgaggcatttgaatggtggtcaaaatgtccaagaaatcattacccatcaacactgtacgtaactgtaagaggactgaaagttccagactgtataaagccatcttaccgctctatgatggctcttcaggaggaaaaaggtaaaccagtgcattgtgaacgtcaccatgagtcaagctcagtagacacagaacctggattagaagagtcaaaggaagtaataaagtggaaacgactccctgggcaggcttgccgtatcccaaacaaacacctcttctcactaaatgcaggagaacgaggatgtttttgtcttgatttctcccacaatggaagaatattagcagcagcttgtgccagccgggatggatatccaattattttatatgaaattccttctggacgtttcatgagagaattgtgtggccacctcaatatcatttatgatctttcctggtcaaaagatgatcactacatccttacttcatcatctgatggcactgccaggatatggaaaaatgaaataaacaatacaaatactttcagagttttacctcatccttcttttgtttacacggctaaattccatccagctgtaagagagctagtagttacaggatgctatgattccatgatacggatatggaaagttgagatgagagaagattctgccatattggtccgacagtttgacgttcacaaaagttttatcaactcactttgttttgatactgaaggtcatcatatgtattcaggagattgtacaggggtgattgttgtttggaatacctatgtcaagattaatgatttggaacattcagtgcaccactggactataaataaggaaattaaagaaactgagtttaagggaattccaataagttatttggagattcatcccaatggaaaacgtttgttaatccataccaaagacagtactttgagaattatggatctccggatattagtagcaaggaagtttgtaggagcagcaaattatcgggagaagattcatagtactttgactccatgtgggacttttctgtttgctggaagtgaggatggtatagtgtatgtttggaacccagaaacaggagaacaagtagccatgtattctgacttgccattcaagtcacccattcgagacatttcttatcatccatttgaaaatatggttgcattctgtgcatttgggcaaaatgagccaattcttctgtatatttacgatttccatgttgcccagcaggaggctgaaatgttcaaacgctacaatggaacatttccattacctggaatacaccaaagtcaagatgccctatgtacctgtccaaaactaccccatcaaggctcttttcagattgatgaatttgtccacactgaaagttcttcaacgaagatgcagctagtaaaacagaggcttgaaactgtcacagaggtgatacgttcctgtgctgcaaaagtcaacaaaaatctctcatttacttcaccaccagcagtttcctcacaacagtctaagttaaagcagtcaaacatgctgaccgctcaagagattctacatcagtttggtttcactcagaccgggattatcagcatagaaagaaagccttgtaaccatcaggtagatacagcaccaacggtagtggctctttatgactacacagcgaatcgatcagatgaactaaccatccatcgcggagacattatccgagtgtttttcaaagataatgaagactggtggtatggcagcataggaaagggacaggaaggttattttccagctaatcatgtggctagtgaaacactgtatcaagaactgcctcctgagataaaggagcgatcccctcctttaagccctgaggaaaaaactaaaatagaaaaatctccagctcctcaaaagcaatcaatcaataagaacaagtcccaggacttcagactaggctcagaatctatgacacattctgaaatgagaaaagaacagagccatgaggaccaaggacacataatggatacacggatgaggaagaacaagcaagcaggcagaaaagtcactctaatagagta

SEQ ID NO: 338 - DNA, 1677 bp, synthetic construct
  misc_feature 1..1677: note = synthesized sequence
  source 1..1677: mol_type = other DNA
atggctcaagattcagtagatctttcttgtgattatcagttttggatgcagaagctttctgtatgggatcaggcttccactttggaaacccagcaagacacctgtcttcacgtggctcagttccaggagttcctaaggaagatgtatgaagccttgaaagagatggattctaatacagtcattgaaagattccccacaattggtcaactgttggcaaaagcttgttggaatccttttattttagcatatgatgaaagccaaaaaattctaatatggtgcttatgttgtctaattaacaaagaaccacagaattctggacaatcaaaacttaactcctggatacagggtgtattatctcatatactttcagcactcagatttgataaagaagttgctcttttcactcaaggtcttgggtatgcacctatagattactatcctggtttgcttaaaaatatggttttatcattagcgtctgaactcagagagaatcatcttaatggatttaacactcaaaggcgaatggctcccgagcgagtggcgtccctgtcacgagtttgtgtcccacttattaccctgacagatgttgaccccctggtggaggctctcctcatctgtcatggacgtgaacctcaggaaatcctccagccagagttctttgaggctgtaaacgaggccattttgctgaagaagatttctctccccatgtcagctgtagtctgcctctggcttcggcaccttcccagccttgaaaaagcaatgctgcatctttttgaaaagctaatctccagtgagagaaattgtctgagaaggatcgaatgctttataaaagattcatcgctgcctcaagcagcctgccaccctgccatattccgggttgttgatgagatgttcaggtgtgcactcctggaaaccgatggggccctggaaatcatagccactattcaggtgtttacgcagtgctttgtagaagctctggagaaagcaagcaagcagctgcggtttgcactcaagacctactttccttacacttctccatctcttgccatggtgctgctgcaagaccctcaagatatccctcggggacactggctccagacactgaagcatatttctgaactgctcagagaagcagttgaagaccagactcatgggtcctgcggaggtccctttgagagctggttcctgttcattcacttcggaggatgggctgagatggtggcagagcaattactgatgtcggcagccgaaccccccacggccctgctgtggctcttggccttctactacggcccccgtgatgggaggcagcagagagcacagactatggtccaggtgaaggccgtgctgggccacctcctggcaatgtccagaagcagcagcctctcagcccaggacctgcagacggtagcaggacagggcacagacacagacctcagagctcctgcacaacagctgatcaggcaccttctcctcaacttcctgctctgggctcctggaggccacacgatcgcctgggatgtcatcaccctgatggctcacactgctgagataactcacgagatcattggctttcttgaccagaccttgtacagatggaatcgtcttggcattgaaagccctagatcagaaaaactggcccgagagctccttaaagagctgcgaactcaagtctag

SEQ ID NO: 339 - DNA, 3825 bp, synthetic construct
  misc_feature 1..3825: note = synthesized sequence
  source 1..3825: mol_type = other DNA
atgcctgagccggggaagaagccagtctcagcttttagcaagaagccacggtcagtggaagtggccgcaggcagccctgccgtgttcgaggccgagacagagcgggcaggagtgaaggtgcgctggcagcgcggaggcagtgacatcagcgccagcaacaagtacggcctggccacagagggcacacggcatacgctgacagtgcgggaagtgggccctgccgaccagggatcttacgcagtcattgctggctcctccaaggtcaagttcgacctcaaggtcatagaggcagagaaggcagagcccatgctggcccctgcccctgcccctgctgaggccactggagcccctggagaagccccggccccagccgctgagctgggagaaagtgccccaagtcccaaagggtcaagctcagcagctctcaatggtcctacccctggagcccccgatgaccccattggcctcttcgtgatgcggccacaggatggcgaggtgaccgtgggtggcagcatcaccttctcagcccgcgtggccggcgccagcctcctgaagccgcctgtggtcaagtggttcaagggcaaatgggtggacctgagcagcaaggtgggccagcacctgcagctgcacgacagctacgaccgcgccagcaaggtctatctgttcgagctgcacatcaccgatgcccagcctgccttcactggcagctaccgctgtgaggtgtccaccaaggacaaatttgactgctccaacttcaatctcactgtccacgaggccatgggcaccggagacctggacctcctatcagccttccgccgcacgagcctggctggaggtggtcggcggatcagtgatagccatgaggacactgggattctggacttcagctcactgctgaaaaagagagacagtttccggaccccgagggactcgaagctggaggcaccagcagaggaggacgtgtgggagatcctacggcaggcacccccatctgagtacgagcgcatcgccttccagtacggcgtcactgacctgcgcggcatgctaaagaggctcaagggcatgaggcgcgatgagaagaagagcacagcctttcagaagaagctggagccggcctaccaggtgagcaaaggccacaagatccggctgaccgtggaactggctgaccatgacgctgaggtcaaatggctcaagaatggccaggagatccagatgagcggcagcaagtacatctttgagtccatcggtgccaagcgtaccctgaccatcagccagtgctcattggcggacgacgcagcctaccagtgcgtggtgggtggcgagaagtgtagcacggagctctttgtgaaagagccccctgtgctcatcacgcgccccttggaggaccagctggtgatggtggggcagcgggtggagtttgagtgtgaagtatcggaggagggggcgcaagtcaaatggctgaaggacggggtggagctgacccgggaggagaccttcaaataccggttcaagaaggacgggcagagacaccacctgatcatcaacgaggccatgctggaggacgcggggcactatgcactgtgcactagcgggggccaggcgctggctgagctcattgtgcaggaaaagaagctggaggtgtaccagagcatcgcagacctgatggtgggcgcaaaggaccaggcggtgttcaaatgtgaggtctcagatgagaatgttcggggtgtgtggctgaagaatgggaaggagctggtgcccgacagccgcataaaggtgtcccacatcgggcgggtccacaaactgaccattgacgacgtcacacctgccgacgaggctgactacagctttgtgcccgagggcttcgcctgcaacctgtcagccaagctccacttcatggaggtcaagattgacttcgtacccaggcaggaacctcccaagatccacctggactgcccaggccgcataccagacaccattgtggttgtagctggaaataagctacgtctggacgtccctatctctggggaccctgctcccactgtgatctggcagaaggctatcacgcaggggaataaggccccagccaggccagccccagatgccccagaggacacaggtgacagcgatgagtgggtgtttgacaagaagctgctgtgtgagaccgagggccgggtccgcgtggagaccaccaaggaccgcagcatcttcacggtcgagggggcagagaaggaagatgagggcgtctacacggtcacagtgaagaaccctgtgggcgaggaccaggtcaacctcacagtcaaggtcatcgacgtgccagacgcacctgcggcccccaagatcagcaacgtgggagaggactcctgcacagtacagtgggagccgcctgcctacgatggcgggcagcccatcctgggctacatcctggagcgcaagaagaagaagagctaccggtggatgcggctgaacttcgacctgattcaggagctgagtcatgaagcgcggcgcatgatcgagggcgtggtgtacgagatgcgcgtctacgcggtcaacgccatcggcatgtccaggcccagccctgcctcccagcccttcatgcctatcggtccccccagcgaacccacccacctggcagtagaggacgtctctgacaccacggtctccctcaagtggcggcccccagagcgcgtgggagcaggaggcctggatggctacagcgtggagtactgcccagagggctgctcagagtgggtggctgccctgcaggggctgacagagcacacatcgatactggtgaaggacctgcccacgggggcccggctgcttttccgagtgcgggcacacaatatggcagggcctggagcccctgttaccaccacggagccggtgacagtgcaggagatcctgcaacggccacggcttcagctgcccaggcacctgcgccagaccattcagaagaaggtcggggagcctgtgaaccttctcatccctttccagggcaagccccggcctcaggtgacctggaccaaagaggggcagcccctggcaggcgaggaggtgagcatccgcaacagccccacagacaccatcctgttcatccgggccgctcgccgcgtgcattcaggcacttaccaggtgacggtgcgcattgagaacatggaggacaaggccacgctggtgctgcaggttgttgacaagccaagtcctccccaggatctccgggtgactgacgcctggggtcttaatgtggctctggagtggaagccaccccaggatgtcggcaacacggagctctgggggtacacagtgcagaaagccgacaagaagaccatggagtggttcaccgtcttggagcattaccgccgcacccactgcgtggtgccagagctcatcattggcaatggctactacttccgcgtcttcagccagaatatggttggctttagtgacagagcggccaccaccaaggagcccgtctttatccccagaccaggcatcacctatgagccacccaactataaggccctggacttctccgaggccccaagcttcacccagcccctggtgaaccgctcggtcatcgcgggctacactgctatgctctgctgtgctgtccggggtagccccaagcccaagatttcctggttcaagaatggcctggacctgggagaagacgcccgcttccgcatgttcagcaagcagggagtgttgactctggagattagaaagccctgcccctttgacgggggcatctatgtctgcagggccaccaacttacagggcgaggcacggtgtgagtgccgcctggaggtgcgagtgcctcagtga

SEQ ID NO: 340 - DNA, 1110 bp, synthetic construct
  misc_feature 1..1110: note = synthesized sequence
  source 1..1110: mol_type = other DNA
atgttgaagccatcattaccattcacatccctcttattcctgcagctgcccctgctgggagtggggctgaacacgacaattctgacgcccaatgggaatgaagacaccacagctgatttcttcctgaccactatgcccactgactccctcagtgtttccactctgcccctcccagaggttcagtgttttgtgttcaatgtcgagtacatgaattgcacttggaacagcagctctgagccccagcctaccaacctcactctgcattattggtacaagaactcggataatgataaagtccagaagtgcagccactatctattctctgaagaaatcacttctggctgtcagttgcaaaaaaaggagatccacctctaccaaacatttgttgttcagctccaggacccacgggaacccaggagacaggccacacagatgctaaaactgcagaatctggtgatcccctgggctccagagaacctaacacttcacaaactgagtgaatcccagctagaactgaactggaacaacagattcttgaaccactgtttggagcacttggtgcagtaccggactgactgggaccacagctggactgaacaatcagtggattatagacataagttctccttgcctagtgtggatgggcagaaacgctacacgtttcgtgttcggagccgctttaacccactctgtggaagtgctcagcattggagtgaatggagccacccaatccactgggggagcaatacttcaaaagagaatcctttcctgtttgcattggaagccgtggttatctctgttggctccatgggattgattatcagccttctctgtgtgtatttctggctggaacggacgatgccccgaattcccaccctgaagaacctagaggatcttgttactgaataccacgggaacttttcggcctggagtggtgtgtctaagggactggctgagagtctgcagccagactacagtgaacgactctgcctcgtcagtgagattcccccaaaaggaggggcccttggggaggggcctggggcctccccatgcaaccagcatagcccctactgggcccccccatgttacaccctaaagcctgaaacctga

SEQ ID NO: 341 - DNA, 151 bp, synthetic construct
  misc_feature 1..151: note = Synthesized sequence
  source 1..151: mol_type = other DNA
gggtgatgggtgctggccaggacacccactgtatgattgctgtccaacacagccccagcctttgagacctctgcccagagttgttctccatccaacagggccatgagccccatgactgtgagtactggctttcgcagcaactgcacatggg

SEQ ID NO: 342 - DNA, 151 bp, synthetic construct
  misc_feature 1..151: note = Synthesized sequence
  source 1..151: mol_type = other DNA
actacagttgctccgatatttaggctacgtcaataggcactaacttattggcgctggtgaacggacttcctctcgagtaccagaagatgactacaaaactcctttccattgcgagtatcggagtctggctcagtttggccagggaggcact

SEQ ID NO: 343 - RNA, 71 nt, synthetic construct
  misc_feature 1..71: note = Synthesized sequence
  source 1..71: mol_type = other RNA
gtcaaggcactcttgcctacgccaccagctccaaccaccacaagtttatattcagtcattttcagcaggcc

SEQ ID NO: 344 - RNA, 81 nt, synthetic construct
  source 1..81: mol_type = other RNA
ggaggcagcggcggaggaggcagcgcctgctcgcgatgctagagggctctgccagtgagcaagggcgaggagctgttcacc

SEQ ID NO: 345 - RNA, 70 nt, synthetic construct
  source 1..70: mol_type = other RNA
ccgcctcctccgtcgcggacgagcgctacgacctcccgagacggtctctcgttcccgctcctcgacaagt

SEQ ID NO: 346 - RNA, 151 nt, synthetic construct
  source 1..151: mol_type = other RNA
cggcgcccgccgcccgcccggagcccgcgagcaaccccagtcccccccacccgcgcgtggcggcgccggctccctagccaccgcggccccaccctcttccggcctcagctgtccgggctgctttcgcctccgcctgtggatgctgcgcctc

SEQ ID NO: 347 - RNA, 111 nt, synthetic construct
  source 1..111: mol_type = other RNA
gctcccaggtgcgggagagaggcctgctgaaaatgactgaatataaacttgtggtagttggagctggtggcgtaggcaagagtgccttgacgatacagctaattcagaatc

SEQ ID NO: 348 - DNA, 43 bp, synthetic construct
  misc_feature 1..43: note = Synthesized sequence
  source 1..43: mol_type = other DNA
ccacctgttcattacaatggcccctcaaaatgaaaatggccag

SEQ ID NO: 349 - DNA, 60 bp, synthetic construct
  misc_feature 1..60: note = Synthesized sequence
  source 1..60: mol_type = other DNA
ccacctgttcattacaatggcccctcaaaagcagggtatgttgactttgaaaatggccag

SEQ ID NO: 350 - DNA, 61 bp, synthetic construct
  misc_feature 1..61: note = Synthesized sequence
  source 1..61: mol_type = other DNA
ccacctgttcattacaatggcccctcaaaaagcagggtatgttgactttgaaaatggccag

SEQ ID NO: 351 - DNA, 39 bp, synthetic construct
  misc_feature 1..39: note = Synthesized sequence
  source 1..39: mol_type = other DNA
agcgcctgctcgcgatgctagagggctctgccagtgagc

SEQ ID NO: 352 - RNA, 75 nt, synthetic construct
  source 1..75: mol_type = other RNA
agcggcggaggaggcagcgcctgctcgcgatgctagagggctctgccagtgagcaagggcgaggagctgttcacc

SEQ ID NO: 353 - RNA, 47 nt, synthetic construct
  source 1..47: mol_type = other RNA
cgctacgacctcccgagacggtcactcgttcccgctcctcgacaagt

SEQ ID NO: 354 - RNA, 40 nt, synthetic construct
  source 1..40: mol_type = other RNA
cgctacgacctcccgagacggtcactcgttcccgctcctc

SEQ ID NO: 355 - RNA, 35 nt, synthetic construct
  source 1..35: mol_type = other RNA
cgacctcccgagacggtcactcgttcccgctcctc

SEQ ID NO: 356 - RNA, 28 nt, synthetic construct
  source 1..28: mol_type = other RNA
cgacctcccgagacggtcactcgttccc

SEQ ID NO: 357 - RNA, 22 nt, synthetic construct
  source 1..22: mol_type = other RNA
cgacctcccgagacggtcactc

SEQ ID NO: 358 - RNA, 15 nt, synthetic construct
  source 1..15: mol_type = other RNA
cgacctcccgagacg

SEQ ID NO: 359 - DNA, 39 bp, synthetic construct; identical to SEQ ID NO: 351
  misc_feature 1..39: note = Synthesized sequence
  source 1..39: mol_type = other DNA

SEQ ID NO: 360 - RNA, 78 nt, synthetic construct
  source 1..78: mol_type = other RNA
ggcagcggcggaggaggcagcgcctgctcgcgatgctagagggctctgccagtgagcaagggcgaggagctgttcacc

SEQ ID NO: 361 - RNA, 71 nt, synthetic construct
  source 1..71: mol_type = other RNA
gtcgccgcctcctccgtcgcggacgagcgctacgacctcccgagacggtcactcgttcccgctcctcgaca

SEQ ID NO: 362 - RNA, 78 nt, synthetic construct
  source 1..78: mol_type = other RNA
ggaggcagcagaaggtatacacgccggaagaatctgtagagatccccggtcgccaccgtgagcaagggcgaggagctg

SEQ ID NO: 363 - RNA, 71 nt, synthetic construct
  source 1..71: mol_type = other RNA
tccgtcgtcttccatatgtgcggccttcttagacacctctaggggccagcggtggcactcgttcccgctcc

SEQ ID NO: 364 - RNA, 112 nt, synthetic construct
  source 1..112: mol_type = other RNA
atggacgagctgtacaagctgcagggcggaggaggcagcgcctgctcgcgatgcnanagggctctgccagtgagcaagggcgaggagctgttcaccggggtggtgcccatcc

SEQ ID NO: 365 - RNA, 111 nt, synthetic construct
  source 1..111: mol_type = other RNA
tacctgctcgacatgttcgacgtcccgcctcctccgtcgcggacgagcgctacgncntcccgagacggtcactcgttcccgctcctcgacaagtggccccaccacgggtag

SEQ ID NO: 366 - RNA, 151 nt, synthetic construct; identical to SEQ ID NO: 346
  source 1..151: mol_type = other RNA

SEQ ID NO: 367 - RNA, 151 nt, synthetic construct
  source 1..151: mol_type = other RNA
gcggggccagaggctcagcggctcccaggtgcgggagagaggcctgctgaaaatgactgaatataaacttgtggtagttggagctggtggcgtaggcaagagtgccttgacgatacagctaattcagaatcattttgtggacgaatatgat

SEQ ID NO: 368 - RNA, 151 nt, synthetic construct
  source 1..151: mol_type = other RNA
ggattacccaagacagagcatcaaagaaacaccttgctggattgaaattcacttacaccgggccctccagctcctagacgaagtacttcataccatgccgattgcagacccacaacctttagactgaggtcttttaccgttggggccctta

SEQ ID NO: 369 - RNA, 151 nt, synthetic construct
  source 1..151: mol_type = other RNA
ctgcggaggtccctttgagagctggttcctgttcattcacttcggaggatgggctgagatggtggcagagcaattactgatgtcggcagccgaaccccccacggccctgctgtggctcttggccttctactacggcccccgtgatgggagg

SEQ ID NO: 370 - RNA, 29 nt, synthetic construct
  source 1..29: mol_type = other RNA
gcccggagcccgcgggcaccccgagtccc

SEQ ID NO: 371 - RNA, 29 nt, synthetic construct
  source 1..29: mol_type = other RNA
cgggcctcgggcgctcgttggggtcaggg

SEQ ID NO: 372 - RNA, 24 nt, synthetic construct
  source 1..24: mol_type = other RNA
gatgttggcagccgaaccacccac

SEQ ID NO: 373 - RNA, 24 nt, synthetic construct
  source 1..24: mol_type = other RNA
ctacagccgtcggcttggggggtg

SEQ ID NO: 374 - RNA, 24 nt, synthetic construct
  source 1..24: mol_type = other RNA
ttcctgttcattcactttggaaga

SEQ ID NO: 375 - RNA, 24 nt, synthetic construct
  source 1..24: mol_type = other RNA
aaggacaagtaagtgaagcctcct

SEQ ID NO: 376 - RNA, 24 nt, synthetic construct
  source 1..24: mol_type = other RNA
cctcccatggccctgctgtggctc

SEQ ID NO: 377 - RNA, 24 nt, synthetic construct
  source 1..24: mol_type = other RNA
ggggggtgccgggacgacaccgag

SEQ ID NO: 378 - RNA, 111 nt, synthetic construct
  source 1..111: mol_type = other RNA
ttgccgtcccaagcaatggatgatttgatgctgtccccggacgatattgaacaatagttcactgaagacccaggtccagatgaagctcccagaatgccagaggctgctccc

SEQ ID NO: 379 - RNA, 111 nt, synthetic construct; identical to SEQ ID NO: 378
  source 1..111: mol_type = other RNA

SEQ ID NO: 380 - RNA, 121 nt, synthetic construct
  source 1..121: mol_type = other RNA
ccgctagaaactgcagagacctgaaattctgccatcctgaactcaagagtggagaatactaggttgaccctaaccaaggatgcaaattggatgctatcaaggtattctgtaatatggaaac

SEQ ID NO: 381 - RNA, 111 nt, synthetic construct
  source 1..111: mol_type = other RNA
tctttgacgtctctggactttaagacggtaggacttgagttctcacctcttatgacccaactgggattggttcctacgtttaacctacgatagttccataagacattatac

SEQ ID NO: 382 - RNA, 121 nt, synthetic construct
  source 1..121: mol_type = other RNA
tgatggagtactatcccaatggatctttatgcaagtatttaagtctccacacaagtgactaggtaagctcttgccgtcttgctcattctgttactagaggactggcttatcttcacacaga

SEQ ID NO: 383 - RNA, 111 nt, synthetic construct
  source 1..111: mol_type = other RNA
ctcatgatagggttacctagaaatacgttcataaattcagaggtgtgttcactgacccattcgagaacggcagaacgagtaagacaatgatctcctgaccgaatagaagtg

SEQ ID NO: 384 - RNA, 121 nt, synthetic construct
  source 1..121: mol_type = other RNA
tccatccagctgtaagagagctagtagttacaggatgctatgattccatgatacggatatagaaagttgagatgagagaagattctgccatattggtccgacagtttgacgttcacaaaag

SEQ ID NO: 385 - RNA, 111 nt, synthetic construct
  source 1..111: mol_type = other RNA
ggtcgacattctctcgatcatcaatgtcctacgatactaaggtactatgcctatacctttcaactctactctcttctaagacggtataaccaggctgtcaaactgcaagtg

SEQ ID NO: 386 - RNA, 121 nt, synthetic construct
  source 1..121: mol_type = other RNA
tgatcaggcaccttctcctcaacttcctgctctgggctcctggaggccacacgatcgcctaggatgtcatcaccctgatggctcacactgctgagataactcacgagatcattggctttct

SEQ ID NO: 387 - RNA, 111 nt, synthetic construct
  source 1..111: mol_type = other RNA
tccgtggaagaggagttgaaggacgagacccgaggacctccggtgtgctagcggaccctacagtagtgggactaccgagtgtgacgactctattgagtgctctagtaaccg

SEQ ID NO: 388 - RNA, 121 nt, synthetic construct
  source 1..121: mol_type = other RNA
ggggtcttaatgtggctctggagtggaagccaccccaggatgtcggcaacacggagctctaggggtacacagtgcagaaagccgacaagaagaccatggagtggttcaccgtcttggagca

SEQ ID NO: 389 - RNA, 111 nt, synthetic construct
  source 1..111: mol_type = other RNA
gaattacaccgagacctcaccttcggtggggtcctacagccgttgtgcctcgagacccccatgtgtcacgtctttcggctgttcttctggtacctcaccaagtggcagaac

SEQ ID NO: 390 - RNA, 121 nt, synthetic construct
  source 1..121: mol_type = other RNA
aacgctacacgtttcgtgttcggagccgctttaacccactctgtggaagtgctcagcattagagtgaatggagccacccaatccactgggggagcaatacttcaaaagagaatcctttcct

SEQ ID NO: 391 - RNA, 111 nt, synthetic construct
  source 1..111: mol_type = other RNA
atgtgcaaagcacaagcctcggcgaaattgggtgagacaccttcacgagtcgtaacctcacttacctcggtgggttaggtgaccccctcgttatgaagttttctcttagga

SEQ ID NO: 392 - RNA, 111 nt, synthetic construct
  source 1..111: mol_type = other RNA
gagcccgcgagcaaccccagtcccccccacccgcgcgtggcggcgccggctccctagccaccgcggccccaccctcttccggcctcagctgtccgggctgctttcgcctcc

SEQ ID NO: 393 - RNA, 111 nt, synthetic construct
  source 1..111: mol_type = other RNA
ctcgggcgctcgttggggtcagggggggtgggcgcgcaccgccgcggccgagggaccggtggcgccggggtgggagaaggccggagtcgacaggcccgacgaaagcggacc

SEQ ID NO: 394 - RNA, 111 nt, synthetic construct
  source 1..111: mol_type = other RNA
aagccggtgctcacggccatggggctgctggcgctgctggatgaggagcagctctaggccgaagtgtcgcaggccgggaccgtcctggacagcaaccacacggtgggcgtc

SEQ ID NO: 395 - RNA, 111 nt, synthetic construct
  source 1..111: mol_type = other RNA
ttcggccacgagtgccggtaccccgacgaccgcgacgacctactcctcgtcgagacccggcttcacagcgtccggccctggcaggacctgtcgttggtgtgccacccgcag

SEQ ID NO: 396 - RNA, 111 nt, synthetic construct
  source 1..111: mol_type = other RNA
caacgaccccacgcggcgacggcccccccccgccccgcagatgaggagcagctctaggccgaagtgtcgcaggccgggaccgtcctggacagcaaccacacggtgggcgtc

SEQ ID NO: 397 - RNA, 111 nt, synthetic construct
  source 1..111: mol_type = other RNA
gttgctggggtgcgccgctgccgggggggggcggggcgtctactcctcgtcgagacccggcttcacagcgtccggccctggcaggacctgtcgttggtgtgccacccgcag

SEQ ID NO: 398 - RNA, 31 nt, synthetic construct
  source 1..31: mol_type = other RNA
caaaatcaggggaagtaaaaaccccaccagg

SEQ ID NO: 399 - protein, 13 aa, synthetic construct
  REGION 1..13: note = Synthesized sequence
GGSGGGGSACSRC

SEQ ID NO: 400 - protein, 13 aa, synthetic construct
  REGION 1..13: note = Synthesized sequence
ELFTVSKGEELFT